European Patent Application EP 4 667 941 A1, published December 24, 2025. Title: 콧물 시료를 이용한 반려동물의 인지 장애 진단용 조성물. Applicant: 주식회사 키베이직. The sequence listing filed with the application follows.

SEQUENCE LISTING (4 sequences)

SEQ ID NO: 1 - DNA, 79824 bp, Homo sapiens
  source 1..79824: mol_type = genomic DNA
gtcagagttcgcaactcgagcgcccagagggctcgcgaaaagtcccagcctgcaagccaacctcgctcagcggacgactggccggatcccaacgcgctgccccttgcccagcctgcgagcgcgtggtacgaaggcgcgtctgcatccatgccccagcccggggagctggaggcgctcgcagtcagaggcgagtgatgctaggctgagcgcgtggcggcccgtgtcgtgccccgctgagccaagtgcggaagggcagcggcgcgctccgactctgctcgccgcacgcagggcggggcgcggctggggggcggggggcctggccgcccgctgggagctgcggacgagcaggcgcgctgaggacccgagggaggacacggttaaagcattgctatcaactgtgaacccagagagccctccttagccaacacgctaactccgaagcctcccttacgcccccgaaccaccgaaggcggcgacacctgattcagcgcacaaacacaggtcccttctgtcccggatacaattacgcggcagacacacactcaaactcgcgcggggcagccaagagacgaggtgagcggagggaccacgccgttccagagggcggaagggggggcggtctgggtggaggagaggggcgttgtttgctccctgaggtgagtgccgggcgaatggctgctgtccaggggcgggggggtgggaattagaaagcacagacagggttgggctgaggaagttagaagtggttagtgggggttggcggggtagggagaaaggctaggggttgagggggtgtgaaggagatctttttaggctggcccctcatagcgcccgcgatcctgtttctgccatatggcatccgttcgagggttctctcgcgtttgtgcgctcaaggcagagggagggtataacggggaggcgattcggccgaggaccttgtacttgacccctgaagggatgggcaccgcggagcccagaggccagagccagctgccagggcagggatggaggtgggggaccaggaggagcttcgggacctcttcaactcccctttactccgtcttccccctaaggaggaacaagagcgggatgtgttgggggtggggaatgtcttggggctgtacaagctcgctgagacttttcggggcccgccgtttccgcgtgcccgcgcgactctcgacaatggacagtgtacagtggtggcagggtttcacgggtccccgcgccgatttgggaatggtacggggtgcccttgcattagagaagcctgtgcgggcccccgggattagagaagaggtgagcgcctgcgggcggggagagaaggacgcgctgctggcaaaaagaagggcgccttccatggactggaggagcggcgagggagcctggtatgtgtgttttggatttgaaggaggcaaaccgcatcggagagtgcaagtagatgcagtgcgtcggggcaaaaggacaatctgaggaggtgggcggggtacccaatctctatatacaagctttctggtttaattgagggtttataaaattgagtacggtaaacctgccattgtgcagcacttccttaggaaaggaatagcctctgtacctgtaccgcgagttcccatcacctttcagcatctaggcggggagaggagagaaggtagagaacttctgagagagttctgagaactaacgcgaatggctggattgcgctaactaggcgttcttagcaggaaaatgtcgccaagggaaggagtgggtggcggtatcaaaccaggcgtgctctggagaatcacctttattatgagccagtgttagcagtgacgatagagtcttttatttctggggatcctattggtaaaaattagaaaaaaaccacactactccaaatactccaaaaatcttcagtcccctcaggctgtcaccttgtactaccagtttttcagtatcaatgacgtgaatgttagggagtttggctagatgccaaattgttatcatttctgataatttcatgttcaaaaacgtctatattcactcaaaattggcgtgcttctgacatatccccagaaaaaaatcaccaccatttgaaggaaggatagaaagtgcccttttttcttttcttttttaaaaacttttattttaggttttggggtacatgtgaagggttgttacataggtaaacacatgtcacaggggtttgttttacatattatttcatcactcagttattaagcccagtacccaatggttatctttaaccaatattttaatagtgttaagagtaaccatactttgtccccaggagattttaaaattagagtcatgcatcttaatattatatggtaaaggagaccagaactttgtgttacttgaattaaatcttagccagcttagttttctcctatagaaactgtctcttggtggtttgaggttttgctttaggaatgtgtctgtgttcagcaactcttctagataatgccagagaaaaacactctagtattgtatgatttgcctgccacctacaaggttaagttgacatctagtgttgtgtgacttagtattatacaagtctttaaaaactacaataaagcatagtgccccgatatttagtaaaggcttgatactctattaggaggttgggcataactgaacagaaactatacttctgactttttccaggtaatactactatacaggttcaaactctttttaaatctaagatttccagaggactatgcttgttgtatttaagcttggtacgcgtcttagaataaataaaccaatgcagtaaataaagatgcttatgacaatttttttggataaaaactacttttcgtttaaagattttgacagtttacatttcccaataatttaaattaaaacattttattgcaccttatgaacaactatcagcttcattaccatttaaatattgctaaaaatcccatcttcaatcctcaaatcctttttaaaatcatgcacctgtttatcaaataatatcaatttgttgctttttaattcatactaggattttccaacatacacctgggaatttctaagatatccttggagagtgagaactttgattatttatgcaagatatagtatctcatttatttgacctcatctgcattggtacttatttacataagcacattttctcggtagctgactcttcacaccgtttattactgaaacttaaaaaaaaagagccattataacccacaagcaatttctaaatcttactgtcttccttgttcccttggagaatattggatataagttattctttcttgttgggttgtctttatgaattcataaagaattgaatagtgctattcgctgaggtgtatagagctgtttttgtttatagtaaatggtctcagcctgctgggttgaaatactagaatagagacagaagtaccattcttctttttatgttttttttttttttctgggtcctctttctgttattggctatcactttctgctgctgtcagactgtgagtgggccctgctgctctattatctgttgtctttttttccatcaaatgatgtgggctattgcccgagtgtaaatcctgtagactttgtgacagacactttcagtttacgtgctttatttgtggtttggactgtgaactgaaatgtttaggtttccagaagggtgacctctatataaaaggttttaatgtaccttttatagaaaaaatttgtgtatgagatctttaggagggtgtattaatttcagacaattcagtcttctggaatatcttggtgtttctgagaaactgaagcagcctttaaaaaaaagtttactttcttatgataggcccagatcgtctttgtttaggaatatgtatactagaatattttacatattactttctgccattgaaacttactaactataatgtagtgtagttaatatttttctaccccggaagtccagaataagaagtatgatttgagaatcctgctaaccatacttgaggctacatgaattatttaaatattattttgcaaatctacttatggaggaggtacataatcaaatacatatgattaaaatggtttaatttgatcttgaaaacagtggtaatcatatctccttaatctgaagcatttcacaaacattcattcttttattcaacaaatatttgttaaaagcatactgtgtgccaagcactgtgctctggggatgtgcatacaattaaggccctgggagggctctaggtttaaaagggggagacaaggaggaaacaggctattttcaatatctacagtatagtgctggctgttctgtaagtgccgtgatagagatacacacacagtaccctgagcagaaatttggaagtggtcaattctgtgtggggacaggagatttgagggtttcttagagggtgacataaaagatgaatcactggaggcaggagcaagatcatggagggctgtttgccattctcaggagtatggactattttcagtttaaggttgttttaaacagaggagctatgtgatgagaaaacagctcttacagcaagcaatctagaaggatggatctgaggaatgtgagatttggatggtagtttagaagatattggggtggctttggtaagagaggttgaggtccttgtaccaaagtgttggcagtgggatgaaaaaaaggggtttggttacaacgatattcaggtggtagaacctctaagattaggtgaccaatttggttggaggattgggagtgggtggtataggaggatgggatgggaacttaaaaggagatccagatttgagagcaagagtgatagagttcagttttagacatgtagaacttgaagtgcttatagaaaatcgaactggagatgtgtgtccagtgaatcattgtatgtgagttctgagcacagaggtcctgggctagataggcaggtagataaatggtaggtagataaatggatagacacacagaaacatttaggagttttcagtgtataggtaattataaaccgtgaaagttgataggttttccagggcaagtaccaaaagttaatagggaaacagaggcctggggagatcctaaaatttaagagttgggtagagaaataggaagcaataaagaaaaacgagaaggtacagaacaagagaggcaagaggagagttaggagggtgtaacttttaaaagcagctgaaaactgagaaaatttcagaaagtgagaaggtcaggtactgaaatgagggggtgttagacagtctcggttcccaccccctctcgagccccgaatagctctgtgaccttgagctcacaatttagtttcatttcctcatttagcaaatgaggggagaagcacctactttatagggctactgtgaggatcagatgagataaaatctatcaagcacaatgcctgggaggttactcctttgtgtttaacaaatgctacctgttttatggaaaccaggacttggatttgtgattagaaggtccgtagtcatttttgctttcacaagtactcgctctcagaattcacagagagtgattgaaaatatatttttaagatgaaaatttgatcatacttttaacttttttggttagaggccagtagaatagcagccattgaaagttttgaagggagcagagggagccaactgaacaaaagtccttgaagagagagtggaagttgcctcaagagcgttgcagagatgttgggtttctcaggacaatccatgcttccgccagtcaggagggtctggtggcatatgcattgtgtttaaaaagcacctggtaattaaacctccaggtttctaatgtcttgtttaaagtactcttagtattttaagtgtgttctagttccttagataatctataaggacattgattatacattttagtattagctgaaaataaactcagaaaacaatacagatgatttcaaaatttaacaaaatgtaatttaatatttgatgattccaaaggcacctctatacctcatagggtcttaaaaatcaacatgtgaaaaataattattagcctgtgtaataggggaaggactgatttgtagaggtttgtttgctttttttttttttttcccccaattaagactactatggtaatatttaaatatacctacttttttcctaggattttctgtttggatgaagtgatgctttatattagagattaataaacattttaaattagatttctattttaatatgtgtataagttttttactctgtaattactgcataatttgagaaaatgtttacatctatgcagtggtttggaagtcaaccaacaattgcacatagtacatattgtttactaattggttataaggcatataataaatatttgttgtcccaatacatgtttgttgaataaaacaaaattagatattccatatttttaagatgaaatgaattttatatctgtagttttaatatttaatcatattctttacctgaaaatcgctagccatacttttcgttttcagcacttctctattttgcagttgtgtttcagtgcttttttttttcccactgtgcttagtccttcacgatttatggccctgttatttgtaaagcatagtaatctaagcaggtgattttcagtttaggatttcttctagttccatgttgtatattcaccaagtcagttttagactatatattgtcatgctcagcactcccttacagagataacagatgccaagttgaaattgacttatacagaatgccacacttaggtaagtgtttaggagtgcatagccaaaataaaaatggtacctttggtttatgaatggcagggcatctaggacagtgtaggtcagttcgtattctctggatggacatttatgtaaatattaaaacatttagattagatggaaagatgtatagtaggaacatttcagagatactgtttccttgtagcattgtactatttatctgaattgttaatttggaataatcactatattgattttattttgaagatataatttatttccattgacttgatataaataacagaaatgcatctgcaaggaatccagttcattaaagaaatttacattcgtatctgatttggtaaatatgtgcttgatttgggaatattatataacaaaatatttgtgaaatcattttgtactttttaattgttttgaagaaatttaatactcaaaatatttcaagacaccaaatcatgactttttagttattacattaagctataacttgctttaatgagtaaaaactgtggggctaattttcttccaagtgaaacatcaagtttaaataatgtgcacatgaatttacaaagtagaatcaagtgtgcaaatatgctatatgttctgtaataggttcttgaaaagctgtatataaactcagcttttataagttgagtcatatttatagaataagaaaatagggcaaacatttaacacttcttaaatattaagtgatgggcatacagatgtttgttatgttaatctttatatttttctgtatgttagaaatagtttacagaaaaaaattgtggttagtgacattaaagcacattatatattaaatatactcagggactttgaaatttaaagcaatatcaacatacaatttaccatagaaaaaatcctattctgattttattaatacctgttttgcaaattcagaatttttaatgggtttaattaagcagatacacacacaacaacaacaacaacaaaaaacttggacacacttctgtaacacatcttgaatatagtctcatctgttggaattttttaaacttctacacttaagtcttaatctgattctccctcatcctcataatattcattattcagaggagaggcatcaacaggaagaattcaattttacttaaataaaaattttttactagcaacggaatgagtgattcagtggtggtgtcttcctgctttgagagagctgttctaagactaggcagttagtcttaggcctaagactaggcagttagtctaggggctccacagcaggcccttcctctgggttctctttatgaagaaggcctttgtgttttacatagattttgcatttgtgctgctgtccctattgagttgttctcaccaagccaatctggggagtagctcttaggggaaaactagtcaaacaggtttgcctgtctattcaaaaggagggaagaacggtgaaatgtatggataaaggccaagagtaaaactgttttaagtaatattcatgctaatcactgactgttggttttgaaaatactttgtagacatttgtgagaatgtatcttaatggagataaagtaagagagaaactggaaggggaagtagtttagaagcaggggataaggacaagatggggagaaggaagggaaaaacaatggaggcaaaataagctcaagaaggaaagaatagtgtttcagtgtcatatctgggctttatgtaaactgggtgtgttatagcaggaaaccatggtattgatctgagaatgaatttaattaaaacaaacaaaaaacccccacatgcctgtgatcctcaatgtccaaaatagggagcgtcttgccagggcagggctgaagtttactaggaatattggtgggaaaatgttatagttaaccatctctgatactaatcttatattagagataatacttggtttcccctagtaaagtgttagagtcatacagctttattgtagtttgcaaatctattacacatatatttctactgtttagttctcattctgcccctgaagcatagccctataggtagtagcattttacagctcataacttggtagagtcccaagtaacctttggaagtcaaaatgacaatccagtctggggaatttgatgttaaaactaaagcttcttgcctagaacaagttttggaactatagctcaccacctgcctcatgttctgggaatgctgaaccttgatcccactgaaattacctttaagtagtctttctgtagtcctcagtaatctcctcctttgctccatgcttcttccctgctccttgagagttccttctcctttctcatctgtaatggtaactccccatctgatctttggttgtgcctcttcttccttcctggcatttttattaacatcttttgtcccagcacctctcctcttctctattctcactcctttggtgtagttattcatgcccatagactggatttttatttatatatagatgattcaaaaagctgtatttctaattgtgatttcttctatactctcaagagcttagagttcccagctcaacttcctaactcagatctgacatccccatttgcctcagtcttcgaagacagattttggtgttgtggaattcacttttttaccctttatatctaatctattcctaattgatcactatgtccttcatgaagaccttcttcccttgcctgagtctttccattcacctcctgatgtcttggtgtagtcccacatcacttcttcaccagtggtactaaatgactcattttcaccattacctgggccttccatcacctcctactgcccacaaccatcagtcacttgtccttactgacccacttgccttctttgagtgtgatttgactatgcgtttattttcacatggggatccaaaatttttagcatggctttcgaggctgtctattgtctagctgctttctgatcagacttatttattttctcatattgctcaataggattctatcctgtttacccactggggcattcatttcaggatatccccccgcttgagatgtcctgccttttttttcttctgcacttccaaattctcacccaaggttttgacactcaagtcccacctcagactgtggcttcccagtctctgtcacttttctgtgactttgatttgtacatatattgatgttagcaattaggtttcattctccctctaaggagagtatgaactcttagagggtggagtctcttgtctcctcatacaccttggacaaacactattgatcagagagaagatattcaaacatgattgaatggtatctttagtttgtcatgaggcaataagggtaagtttcctaattttctatacgtattttgattttttcctgttgttttttccagaactgcatcattcaaacttgaaacattcccctatttttttttaacaaggtgttctatataggaacaacatatcttatagggattgctacattatttagtcacaatggaaaaaaaagtttgatatatagaaagattatataatagttacatggaactctactataaaattataatggtttagtgggttttcttttttaaatttacctggggcttctataggtggatgtgcattcacaactaattctaggtaatgctaataaaagaaaataatcacggtgataattaactgtatttagtttttattttgtatttacatttcaatgtaagtatgcctaatgtcatgaaaccatagttggagaaaataatgattatatgcatgaggaagataacttaggaagcattctaattgtccaactccccacttccccatagaccttttataacaattaaatcaaagcaccagcccaggaataattcttttttccattctttgtgcctatttcctcctttgataattgctgaattcttctggtcagaatatctccctttccatctccctctgagcagagcaataggaataggaatatattttaagccaggtgaagtggtgcaggtctgaggtccagctactctggtggctgagatgggaggattgcttgaggtcaggagttgaggctcaggctgtagtgtgctgtggagatcgtgcctatgaatagccattgcactccagcctgggcaacatagtgagaccttgtctcttaaaaaaagaatatattttaagaaaattcctcagctaaagtaaaaagaaaagagagataagctaggtaagattattaatcagaagtaatgcttgtctgtttaatttgccagttttaaataattcttgaaggcatttgagaggtcattatattcttttaatcagttagactttatctgaatatatgctttggaatatactttttcttcaaacttctaaactatgtgcaatatacagaaacaaggtcctctggctgtcctgctttctgcttgctttttttctctccctttcacttttctggagataatttttctgcctcttgtagggaattcagaggagggatcctagtgattggctttacaaatttgtgtgggggagggattggatagagtggagatgggataggcatctgcccatcagtaggatttggttgtttgtccagcctctatatgggctttaaatgctttatactttctgaccattatttttgccagcaaaaatgatgtagcttattttgatactacttaaatgcagtcctgtccttattctacccctactactccatccaaagggagactgaaggggagacattttgaaccagacatgttgatttcctggtggcctgtacagtgagtattttgtaacatttagaattaattcagtcattcatttaataagtaacctaatatatgctagaaatcttctgtcttagagccaaaatatattgtaattttttcatggtctaagtatctaaggctttacagtataaaagtttaataaagtcatgaccaaggctttacaaagactgctattttgattcatgtatcacagaattcaataaaaagtcaaactattatctgacatatggcagtgacaactttggagggtgtttatatggtacaaatagaagatgctggattaggacctaggaaacctgaatgctggttccgactctgccagcgaataactgaactagctgtgtaatgcaaagacaaccaccccatagagactttgcccctttctctacaaatgaggggtttgaaatcacctatctttagtttttaaattgtgactcatttatttaatgaaaatatatggtttttaaaattttgatatcattttggtacaaatatattgtgtcaatgtttaaatatatttatcttattttcacaagacaatggcaatgatatacaaaagactttctctggacttgcctcattgtggtgaatatcggttataatcatagatacttagaagacacaaaattatacattcttacctgttagtaaaggaacatcaaagaaattcattctgtttttctgcagaaactatcaaaatttttccacttctggggattaagataacttctgttttttatctaatactcaacctatctaatacaaccttgtcctagtgatgatggtagaattttataaaatagggaagtttgttatttgttcacctgtgaagaccttcaaggaattgaataggaaaatacctagagttttgtttcttgttctgatttgcttgtttatatttggccagttttgtcctgaaaatatgtttgagagattacatgaaaatttattttgtgactcttaatataaatgttaaaaatacatttaaactagtgatagtaaagaaagaatatcttaattagtgggggaaataatcccatgatcttttgtgattctacaacattactgtagccttaagaatctctactaatgttgtattgaaaagctgtttctcctacatgtgaatatgtttcattgcaggagaagatgaaagtttgatctggatattctccagattcacttgctgtattctactaattaaaatcccaataaaagagaattatgaagagtcctaacaaaacattttaaaatgtcaatcattgtttttgtattttttaaaaataaaacgtatacacgttagactgtaaagccttaatctcagttgtatgatttgtgaaacttttctcacttgtgtaaagatgggatcagaatcaaaacaattaatttccatattgtttgctgaatgtttatcacatgctgcagatgcgtggagataactgtaccaggctagtcttggggaatttcagaaatagaaacccacatctttttctgtaggataacatagccatatatatccatatatatatatatatatatatatatatatatatatatatatacacacacacacagagatattagatatatataatatctatattatatattagatatctatatataagatagccgtatatatccatatatatatatatatatacacacacacagatgttagaagacacaaaactttacattcttacctgtataatcatagatacttggaagacatatattgtagatacttggaagacatagattcttacctgtataatcatagatacttggaagacacatatttacatatatataaatatgtatacatatatatttttaaaatgaggtatgtgatcaagacgaaagttttaataccactgttttctttattaaaaaggaaaattgcattttttaaaaattacaaacttttatccttattgtctaaatttggtttctggaacagaagcatcagtgttacctggtgacttgttaggaatggaaattcttgggctcatcccagatctgtaaaatcagaaaccatgagggcaggccccacatgtgtgtttgaacaagacctccaggtgattgtgatgcctgctgaagtttgagacccacttatctatgataccagatatctcatcaattcacttttctcacataatgaaaaaattctgatcatcttaaggacaaaagaaaaatttagtttagattttaaaatgctttccaggtaagttttataacctaaactcgtatcttattttacttactaattggttattgaggcatcaacaaatattcttagttcagataaacccacacatttctcagtttattaaaaaaaaacagggttgaattagttgtttattttggtatactttgctatgacattgtacaagtgtagcctagattttcttaatttttaatcacagggaataaaggggaggagggtttaaaaaagccaaaaacccttagtcctaggcctcatccccagaaattctgatttgattgaactacattgtagatggcaggttttcaggcatctctatttttccaaagcttcccaggtgattattatgtgcagttggactatagccatacgttcaaagattggcccatctaccacgtataggtccattaaaaaaattgcacattagatctattaggttcttttattattttaagcaaattgtcctttcatctatgtttaatttaaaaatattttcttttccagtacgttattggtattgttgatttgcttaaccatgttattgatcattttattactctttattcagcctcctggttttgctgtaagtccttgcttattcaaaatgcactccaagcaccagtagtcccatattactagagagcttgtttcataaataagtatgatggggccctaccctacgtctactgaaccacaatttacattttaatagtgtccctataaaatgtgtcttcacattaatgatcctctataacttaaaatttaaaatcaaggtaaattctttttcttttcattttgtttcttagaattcattggtttgatcttaactgctttttatgaaccaaagatatcaatctcattaaacctattcttaaaccctttttttcccagtaagttttagaatagtaagggatattttaaattatcaaatttcatagccccacctgacaggtgaagaaaattagggacataaattaaatgacttggactaaattacaaagggtactgatttggggatccatagatgcatgctgcaatcattttatttttcttttcattatgtgtcacttaaaatgatatctttgtaatttaaactacttgaactgtgagctaactgaaaagatagtcttagattaccaagtaccatacatgtccaaaaaacctcaacattttatatatacattaacaattattttaattatctgtctaaattgatcttgataatgcttttctaacatactacttcaaattagtttagaatttaattaattaagtaataatggggaagttgactattaaacaacatgaaaatgaaaggaactactatatgtgtttactacttattaagtactaaaaatagtcatgtgcttctgagagactgctggtactttgtatatagaaatttaaacagaaagttgtttggaattgtttgttctgagttcctgggaatctggggctatgtgcattatatttttctaaattcccaagataattgagctttaattcaggtctcgatagttggatccacattaccttcattgtattacctgtatttctcttatgcacataagtaacgagtgctagatccctatctgtcagttcggtgggagaattgcataaatatccccagctgcttactaaatatgcagattcttgggtttctccctagactccataacagcttatttgctgaggtgactttggaacctgtatttttagtaagtacttgaggtgattcttctggacgccagaatttgaaaacaacttcattaggtgattatatctttgtgttttaaatagttaaatttaatcaccatcatcaggcattaattggatacatactgtgtacaaggtactgagtgcagtctgttgatattcgtattatcttatttttattttctcactatatttttgtttttatcttaccttcctgcttaatgttttcagagaaactccccaggtgggcctaagccagctatcactgataagcgaatagggttgagtttctcattacagcttcaccacctgtactgtagatgtctgaaaagagataactgcagatacttgtgttgaagaagtggtaagtgcaactagcttggaatggtacaacagcaacaacaactgtctttataacctctccttcaagaagaggttcttttgtatttctcttggcactcatgaatgttccaggtgcaaaactgaattttttgagtggtattcctaatggtctcttcctttcatatttcatgtgtgtaaagaaaggtctgcctctgtaatactcgtagagatttctattaatcttatttttcataagatggcatactagtttaaggaatggaatagtaacacaatatttttctttatgctcttttaaatgagtttgttatcaggcaaagcaatattttaaaagcaaaagtgattgtgttagaaattttgaccaaaagcttctgacagggaactttggattaatttatttcattaagtttgtgaaatggaaccaaattccttcttcctttgcattcagcatttttcagttttatttctgcagttaagccgtgggcttctatacaaataaatataatttttctgatggaatgaaaaacattaatttagtaatgtggaggattttgaaaatctagagttacttatatttattaactgctgacagccaaactgagttctctctgtgtaaggttttcactcagattgtactcttaaaggtgccagacttttttttttttttttttttgggcaggtggaagttttaaccaacaacaggtggcctcaattttctgaattctttcttctcctacctcaaatcagtatgttcccattctagtgattttaggggattctttgcttttagtagtttacttgctaatagccaccataaataacttaagattaccaagaattgcctacagatgaaagatacatgtttaaaacgagggctatttaacaaccaagtagatataaagcttagtttttcccagtttgtccacagttaacaactttttttaagctttcttttttttctctcttcacatggtgggatatgagtacattaatttactagatactagatctttgtcaagtttttatactctcagtcttattatctgtaaagtgggagccactttcttgccttcatgtgatctcaatatgaaatgagataatgtttagaaagctggtaatgcagggggaaggcatgtagcaattaaaaacagctgctgtttattgatacttgtatgttaagtcaaagcaatagggtgaccagctcgtccccgtgtgcccaagactttcctagttttagcactgaaaatcccacatcctgggaaacttcccccctccccacccagttctaggcaaaccaggatcctgagtccccctagggcttccgtgacttaggaaaggtagcttagttgcttcacacacaataatttgggcataagcaggcagggctggtgttatggttttgcagtctcaggacccaagtgtctttgttgttacaccttttctggtttataattctgcctgtatggtctaggatgttaatcattaccatgtctcattccagctggcaggaaggtgaaaagtgaaactccaagggcatacattagaaattgcacatagcaattctgcttccgtttcactctcattaagtagaacttatttatgtgactaaaacaagctattagagaggtagagaaaaattgtctttcgtctttttggctatatgccaaactgaagtactccagaccctttttgcctgggtatcaggcagcagaggctgcagaacagcggatattggtgaacagcaaatgttgctgcctgattgttcctctggaagttttgtctcagaggagtacctggccatgtgaggtgtcagtctgcccttactggggggtgcctcccagttaggctagtcgggggtcagggacccagttgaggaggcagtctgcccgttctcagatctccagctgcgttctgggagaaccactactctcttcaaagctgtcagacagggacatttaagtctgcagaggtttctgctgccttttttggggctatgccctgcccccagaggtggagtctacagaggcaggcaggcctccttgagctgcagtgggctccacccagttcgagcttcccggccgccttgtttacctactcaagcctcggcagtggcgggcgcccctcccctagcctcatggccgccttgcagtttgatctcagactgctgtgctagcaatgagtgaggctccatgggcgtaggaccctctgagccatgcgggggatataatctcctggtgtgctgtttgctaagaccgttggaaaagtgcagtattagggtgggagtgacccgattttccaggtgccttctgtcacccctttctttgactaggaaagggaattccctgaccccctgtgcttcccaggtgaggcgatgcctcaccctacttcggctcatgctcggtgtgttgcacccactgtcctgcacccactgtccaacactccccagtgagatgaacccagtacctcagttggaaatgcagaaatcacccgtcttctgcgtcactcatgctgggagctgtaggctggagctgttcctattcggccatcttggctcccatgtatggtattaaactctggtattttagctttagtctctttggaaaaatgggaaatacaggggatttataaaattctattttcatctttaaaatatttcagtagtatattggggtgttcctgtatcaaatttcagcatatatgaaccattgatacctaggcacagaagcattgtagctaatctaacttgttttctggagctctaagggtttaaaacctttcctttgtgctgtgcatggtggctcatgcctgtaatcccagcactttggtaggctgaggcaggcagatcacacggtcaggagttcgagaccagtttgaccaacatggtgaaaccctgtctctactaaaaaaaatacaaaaattagttgggcacggtggtatgtgcctgtaatcccagctactcaggaggctgaggcaggagaattgcttgaacctgggaggtgaaggttgtagtgagctgagattgtgccattgcactctagcctgagctacagagcaagactccatctcaaacaaaacaaacagacaaacccttcctttggccttggagaaatcacttttacagatgaacgttttggatgtgcaccccaatatcctgatatcttactgtttcacccaaattaattcacactgaaatgttaaatgacttccctgtggtgagtggtagacacacctattaaaatgcttttggcttcctctcttgaaagcaagcatagaaataatttttaatagaaagaaaaaagggtagactgataatgcagtttgtgtagagtcttcaaatatttgtacattctttgaattttggattttcttcaagattctggcagcatgttactccactgccagaatcttgtagtcaaatagtagtagtatcctagaagccaaaagagaatttagagaaagagagaatcactagtggctactgttaaatggaagtccaaacagataagtggaaaatgggcatttgtatgaattttgggaagcgttagtgcccttaacagtaagaatttggttagaattgtggtggattcaaaggctgacagtaaacatctggggagtaagtggagaccagcaaatagagactgatgttttaagatgcttaactccaaaggaaggatgagagtaaggctccagctccagggatgtgccagctgaaagctgtagaattacctacttttggtagaaatctttgaaaatcctgaaaaatataagaaaaggaaagaaaattgttcaagtccataaccttaaaattgttatcagtttcatctttactttgttatcattataatcactttatatatacatatatatcatatacataattttatttctgatcttcttagtgttatgttacaagtattttctgatattaaaattattttcaaacattatttttgaagttctataattttccatgataaaaatatagtgtaattaaattaatctactgttggctttatagtggtttctggctgtttgctgttggctatgaatgcaatggacatttttctacataagtattggtatctctgtagtgttataaaataatatgccagttgtatttcataacatttacaccagtttacattttcaccaacttcttaagactacactgtgcctttgcaagagttgagcattatcactaaaaataacatccttgccggttttataagagacaagtctaatttgttcatttgttcagtcattccactgtagccctgtcaatgcctcataccacttttcagaactcatgtgtatttattttcttttatattcttcactcaaatttccagtggagcttcgggagaaaaggaatggaaacacttgttttaatctgccattttaaactggaaacctctgcttgctccagatgttctaaacattccaaaaatattaatgattgtgcatttaaatctaatatttgtaaaagcaattgtttgctttgctttatgcttatttttttctctttccagataatcctttaaagctaaacatttttaatggatttatctaaaaacttttaacactgtgctattcaatttactttaaggaaggtttaaggtaaaaaatatagtgattttatttttcaaatataaagcaaatttttaacactattgaataagtttttctttcctcatctatttgtggtacttccttcgtcatctattaggcttatatttattcagggaattccaataggcttcctacactgatgcattgatttcatgtagaattcttgggctaattccagtttttaattattgggttttaaaatatgttttaagatttatatggatatcccaaatcattactgtttctttttcaaaaatgtattctctcttctttttatatttttccaatgaacataggtataattttgattaaatttcgaacaaaacccaacaatcatccagtgggatttggaagaaatgtatcagtctatttataacatgggaaggattaacttttagaatattttcttttgtgaaaacaaaagtgtttctatacatttagaaaatattcctgtgtatatatcttcaggggaagtctggccatgttacaggcaacaaatattctatgttggtaatgtaaaaggtatattgtacactttattgttattgtgaatgaagtattttttcatcatatgttactttaaaataatatttatttttatttcagtgagagtaacacatgcgcactgtggattcctttgtgaatacataaaaggaaaagttaaaactcttataattcacactatccagagaaaaacaatactattttggcaagtatcattcccatatgtgtacacatgtatatattttgcaaagtgctacatgatgtttataatgtttagtatcctaattttcagtcaacatttaatcttgaatatcttatgccatattctttttataagatttttctagtggctgcattatatgaatgaatgacagtgtatttaaccaatccccagttgttgagaatttaacataacttcaagatttgcagatggtaataatcctctcctgcactaaatgaaatcaggagaatacttagggaagtgaaatatctattatgtatgttgcaggttgtatttctgagatatcatttgtcattatatttgtttatggtgcatttgatatgtctgcatattttatttgtattgcttagtttgttttctattgagtatttttcaggtttctttaatataaataatattggctattataataacataattatattaaaatataagataattatatcttgacaatgctattctaaaatataagcagttcattaaaaattatgtgatttctttttactttgtagtaattactgaaataaaatattaaaattaaaaaggaagaattaaacaaaagcacagtgaaagcatttgttctctatgatcatttttgttttaagttatttatgatagataaagtagttttaactgtaactgaacagagtgtacctatggtctgctcagctagatccagaacccagtggagagaccagttttctaccattgttccatcatcaagtactcacctctcgaatatgcaagaagtgacagcagtgagcagtagctgctggaatacctacctgttttggcattagtcttatccctggagttcatatttccttgtaaaatatctcatttttccttcttcagatttgtgagaaggcaacattggagagacacataggtgaggcagtacagtagaataaacatttggaaggtttttctaagatcagctccttaattttctttcttcactgatcttgtaattgtagtcaactttactatagaatcagtatcttctccaaagttaattatttttaaagccttataataatgtaagtgacatttatattatatgtttgtaatgtgcattacttttacttattcttaatggtataatttcaactttcaaatagtttgaaacttcccttagagtaggagaggaaaaaagcatctggaaatatatgtattttagagttcaatcttgttattggaagaatctattagttgcctgctattgatttctttacattgcttgtagtgtttgaatgtttagaaggtatagttgttaaaactgcgtttagatgttgggaatttatacaaataggagggttaatgtattctaaggagtaaaaatagatatcaatttggttatatgtgtgttggtgatgtgtgtataaatctattttgagatttttgaaatgtgtccagtttgcatgagcaattgtttagatcttttttctatttgggggtctaatttagagtctaagaattcattatattgaataggttggtgggtgtatttgcacactatatggtccccacgtatagtatatttatctctaaaaacaataaaagacaactttattacacatatctgttaacatgaaaaggtaggagaagtactggccctcaagtgtacaggcatcctctgacttgacatttgcacctgagttaaaggtacaacatagaagtgtggtctgagacataatcattcatcagtcctttttcaataagtatttactgagatccattaaccctcttgagcttttctattaaaagtttctcttttacataatgccctgaaatgcatcagcaaattgacatagattacataaatatagattgctaggacaactatggtatttaggtaaagggaaaatatatgttaaagatcatttttcctctggaaaaaagtcttttctgcagaattaccaaactaccattcaaaataattattttctaaaacaatctttctttggtatgctttgattataactgcaaatgtaaccattgaattaaaatgatttaaataagagacacgtgctgatatacctggaaattaaaaaggtcagctcttcttcctgggattaacattgacattcaattagaagatgaacagatgttccatagatatttcatagatattcttccaaaaagatatattatgtgtcattcagccttatcaaaatgttatttcaaatgtttgaaaatagtttactgattcaattttcttcccaaacagatccatttttaatatatttcagtttatgtcaactttgctttcaattctatacttaaacataattgatctttcaaaaataaagaggtaattagaacaaatatcaggataatttttaatagtgattttttttgtatgttagtgtataatactatagaatgcattctttttttttattattatactttaagttttagggtacatgtgcacaatgtgcaggttagttacatatgtatacatgtgacatactggtgtgctgcgcccactaacttgtcatctagcattaggtatatatcccaatgctatccctcccccctccccccaccccacaacagtccccagagtgtgatgttccccctcctgtgtccatgtgttcccattgttcaattcccacctatgagtgagaatatgcggtgtttggttttttgttcttgcgatggtttactgagaatgatgatttccaatttcatccatgtccctacaaaggacatgaactcatcattttttatggctgcatagtattccatggtgtatatgtgccacattttcttaatccagtctatcattgttggacatttgggttggttccaagtctttgctattgtgaatagtgccgcaataaacatacgtgtgcatgtgtctttatagcagcatgatttatagtcctttgggtatatacccagtaatgggatggctgggttctagatccctgaggaatcgccacattgacttgcacaatggttgaactagtttacagtcccaccaacagtgtaaaagtgttcctatttctccacatcctctccggcacctgttgtttcctgactttttaatgattgccattctaactggtgtgagatgatatctcattgtggttttgatttgcatttctctgatggccagtgatggtgagcattttttcatgtgttttttggctgcataaatgtcttcttttgagaagtgtctgttcatgattttttttttagacaaagtattagatcagatatttttggggaaaaatgctttgtgattgcttgttttgaatggtgagcattgtattttgttttaagttgttttctggttgttattacagctatgaagtcttacactccatatttcattctcctgtggagtgctgttgggatagcgaaggctgccaaaatcatcatcgtgccgccaattatgtttgaaagccatatgtacattttcaagacgctagcctcagccttgcacgagagaggccaccatacagtgttcctcctctctgaaggcagagacatcgccccatctaatcattacagcctccagcgctacccagggatctttaacagtaccacctcagatgctttcctacagtccaagatgcggaatattttctctgggagattgacagcaatcgaactgtttgacatactggatcactatactaagaactgtgacctgatggttggcaaccatgccctgatccagggtctgaagaaagaaaaatttgacctgctgctggtggaccctaatgatatgtgtggatttgtgatagctcatcttttaggggttaaatatgctgtattttcaactggcctttggtatcctgctgaagtgggtgctcctgctccattagcatacgtcccagagtttaactcactcctcacagaccgcatgaacttgctgcaaaggatgaaaaataccggtgtttacctcatttccagattaggggtcagctttctggttcttcccaaatatgaaaggataatgcagaagtacaacctgctgccagagaagtccatgtatgatttggttcatgggtccagcctgtggatgctgtgtactgacgtagcactggaattcccaagacccactctgcctaatgttgtttatgtaggaggaatcctaaccaaaccagccagcccactaccagaagtaaggtttgccgaattccttggtaattcttttttaatgtaaaagtcaattttgatttttggaagagatatgatttgttatttatatatattgtatatatacagtacactaaaaggtgattaggacatggggcctccaaagtccctttatgtgggtccaccacttccctgggaaacattcctgctttgaatgagcatttctgtaatactgaaaagaccactatgccatatggtcaatagactgcctgggaagtagttttctgattaagtaatagttatagtatgtgaggagaatatagttaaatggttaattttaatgagtataagtgattttatctttaattacacacagaatcccctctgttctgccccaaatagcacaattaacaggtatatatgtttagcttcaggtcagtgaacagaggttcttctctgggaggttattaccactagtttatgtccaataatgaaagtgaggtggtaacttccatcaaagtagggagttggttaatttaagctagtaagtaaatgtaatggttttaaggaaagcatgctctattgcaatttcatttcaatgatggaatcaatggcactttaagaaactctgttctctatgtgaaacttaaattctttttattgattgagccaacagtaaatcccttggtattctgttcaccatccttgttttttattaggtatcccacattagcagaagccatacacatacctattgttgtagtgagttttctaacctcagattgaatctctcaatttaacctcaacatcagatcccatttactaggaagtgtagggcttgttgcaggactttattcaagttacttttaatcctacctctggaaatagccactcaaaacaattttgctaaattgttgatttctagttctggtactacatattaaaaattctatcagggccttgatgaagagtaaatccagattttctcgtatagatgaggacaatcacatggctgaattttgtcgtgaggcaataaggtgattagaaatatacgacctgtaggcttttctaatatggccattagagttataattaataaataatatatcgatatatttcatataacatggaaacagaaatggcctgtacacccacagcatttcaaatatatacagccactggaggccatgagggcacacttgttctctctgacgtcaactgtaaaggatagggattaatctcagcttatcttagccattcttgaatttatccaagctcattttgaatcctcagatcttctctggcagagtcaccttcctaaaggtagctaaaatcagattttagaagtagcttctaaaagatttggtaatcaaggtgtgtctttaccttaactgagtcatttaaaatgttacacaaatcatccttgttctctctaggtcatcatcttttccgagctagaacactccccttctgccagctccctttggttttcatctgggtgatgtctctcttcttcagtcacttgattgaagaagaagtatatgatgaaaaggagctggacgcggtgtcccatgcctgtaatcccagcactttgggaggccaaggcaggaggatcacttgagtccaggagttcgagaccagcctggacaacatagtgaaaccttgtctctacaaaaaataaaaattagctgggtatggtgatgcatgtctatagtcccagctactcaggaggctgaggtgggaggatcacttgagttcaggaggtcgaggccgcagtgagctgagatcacaccactacactccagcctaggtgtcagagtgagaccctgtctaaaaaaaaaaaaaaaaaaaaaaaaaggaatgtcctgtcctgattgccttttctttccttccagttcctgctgtatatttgtcttgagttgcagcaacttgaatgacacagtataagtgtaggaaaatattttatgttttattttcaatactctacctttcaaaaagatgcatagcatgtgataattttttttctaccatccaagcatttttttctgtcatggattcctctgcacacagatgtccttactagtgtcactattttgttttacatgaaaaacatctttttagtggtttttggtgctcgacataaggtattactcaaaatatcctttaatttgccataatttctcatttgacactggcttgactttctttgtggagttctttttcctctgggctatttgtagtggttcttttgaaatgcgttttttgtttacaaagtttgctttgtgccagttagtttggttgcatgcacagacatggcatgtgtgcatgtgttatatatagtatgtggacatagataagtatattattattattggaagtctattagattatcattgtgaagggctgttttcatttcagaatgttatttatagtttttgagcagggagtattttgaagaatgatgtgcagtactctttcaggtattccttattctggtgtggttttatatgcttatgaacacatgttcccactgagatttttctagtagatttatttgagataataaactgtaccttttcattctaaaagttaatgagtttctcaaatgcctgtattatttacagggcattgttgtgacagtaacacaggaaggcccagaaagtagctgcgtagaacacatgattcacatatagcagcttaattgttaattgccctggtatcttacactgggcatagattaggttttccagatgtctgtaaatgattttacagtgggactgaatttcacaacctgggatgaaagggcagagaaaatttataaaggacattttaaataagctttcacaatgtttgatcctaaagaaatcctgtagagagcatatagttcggctccattccttttatttattctttcctttaaagtaggtagaatagagatagggaatagtccatccatttctcacatagtagatacaaagacttcatcaaaagccacacagatagtctgtggcaaagtcaggtgtaatgtggattgttttgctatttattaggtgttttttcaaggtgattgcatctcttgtcactaattttagtcatttacttacttacaattgtgtataaaaccatgcagagacagcagttttttgaatcttatttattttatgtctctcaaagattgtcagggcttaatactcaagtcaaatgaaaccatatggactcttatttatgctttagagatttgataaactaaatcagcctaagttcaaatgcttttgattacaaaatgttgtgtcagtgtagagtgaagaaattgtgtgccttgatagtagaaatcattttaaaatccatgttagaaatgtgcctggaaagacaacttatcatctactacctggctgcctctaataggagtctttaaacaatgtggactaaggggaagaattctgagttggatcacattcatatagtggtttacctactctatcattgcaggccagtagagaacatggataaagattaaaaaataaaaatgctttgatcaagaaggaggtctgtagacaggtccctatttgaatagattctttttttttttttttttttgagatggaatctcttgctctgtcacccaggctggagtgcagtggcatgatctcagctcactacaacctctgcctcccaggttcaagtgattctcctgcctcagcctcccaggtagctgggactacagactagtgctaccatacccagctaatttttcgtatttttagtagagatggagtttcaccgtgttagccaggatggtctcgatctcctgaccttgtgatctgcccgtctcggcctcccaaagtgctgggattacaggtgtgagccaccgcgcctggccaaatagatcctttaaatattaaatgtgaatgaaataatgacatctaattggaaagtgattttaatttttattaattttattagcagataatccaccaaagaatagtacatgtttacttagggaatctaatagttattaaaaataaatgtttcaagtgatactttttagatgatttcccattggctgaaatggcctacgctgccaggcagttgctctctgccacttttcaacttctacagccttgaactcttatagcacctaatagcactttaactactgtttgctgttgttgtactgtttttgttgttgtttgtttgttttacatggctctcttaactagaatgtgagtacctcaaaaggttgatactctataacctgagtgcctgaaaaatggttggtactcaataaaactttaatatttaatgaactgtatcaaatagaaatagttgccaaaaataggtgattcagttagtgcaacaatgttaatattataactatcatctgtttgttctaaatttgtgtctgtatactgtcctagccattaagcaacccaaaaatccatgctaagttgttgagttttttttttaatttttattttttgagatggagtctcactctgtcacccaggctgaagtgcagtggcatgatcttggctcactgtagcctctgcctcttgggttcaagcaattctcctgcctcaccctcccaagtagctgggattagaggtgtatgtcaccacgcctagttaatttttatattttcagtagagacagggtttcgatatgttggccaggatggtctcaaactcctgacctcaagtgattcagccaccttggcttctcaaagtgctgggattacaggcatgagccactgccccagctggtactaagttattttaatgaattagaataactattctaatgttactgatagtgaggaaagaagataaccataccattacccaattgtgaactaaaatagtcttttctctcttccaaatatgcatataaacaggggcagtgctgaaagtcaggccagctattgctgtcttgaaagatgatttgaggcagcatggcactcatttggtgctcttcagagatactatatttccacattaggagtatttatggcatcttaagttcaccagttgtggagacatttttatttaaggaagcatagtcttggggagagataagagataaacagagataagaaagcacatgggaccagggactagaccaggagatattcactgtttgtcattttgttatttgctggaactccctcagagaatgatcttggggacaatgagagattgagcaacagagttattagattagccacttgtgagcaggtaagtttatgagaagaaaaatgaaatgaagaaacaaaatagtgactttccatacttggtattcctgattaacatagaagccattacttcctattacatatggtgattgaaagctggtttcaccattaatgaatgaagtctctaggcttggatatgagaccagggtccttgggggtaaaagacttgatccagggttgcagcagatgtggaaaattaaggccatttttattaataattacatatgcaatttgttatcttatgaaatttaaagctggagatgtaaagcttcatctatatagtagtactatgctatgttgttagctatgtgggggtcagaaaattgaggatgacaatgtttagaagagactaataatttcattccagttactaattctgagttcagaaatgttagtactttaactactgtttgtttgtttgttggatggctctcttaactagaatgtgagtacctcaaaaggttggtactctataccctgaatgcctgaaaagtggttggcactcaataaaagtttaatatttaatgaactgttaaatgatagtttggcagaaaaaataaattctctaagggaactcattaatgtaaaatgtttttgcagatgctttataggttaatcatgtattttcttattattttgtagtaagaaaccaaatttatagtaagtaaccaaatttcttgttaaagaaatctatccaggaagtaagtaaatcaagcactgttgaaactatcaatgacttaactgttcagttcactgatacaaaaattttctaagcaacattgtagtttttaatagcttgtcatctgcttctgtaagcattatgggcttacaaggatttcctgatatgataggagatccaatatatgaacggaatcaaacaaacttgttttgaattgatattgcaagatctgacatgattttaactccagcacacattgttaagtttttaagctttaataagccctagagaattgttcatttaggtattaagtcaaatactggcaatatttttaagggaaatatttttaactgataatttttagaaatgacaaatttctcaattaaattactgttgacaccagttttgggggatgatattcttcacaaatactcttattctaagccaaacaggtctatttatgaaatttaaattgctactgccaaagggtttgtcagatctatttctgagctcagattttgtggtgtaagcatgagcttgtgacaaatcagtggcactgaagacaaactacctattttctggctttgtatatgaaaaattgtatttcacctttccaggtattgttccttgtacaaaataccaaaatggaaaaacaggggcttttttagtcaaatggccctgacttttagtcttatcttcatacgactcttttggttaaaggaatcagcctaattaaaatgaggatagcatgtcagtacttacttcagaggacttttggtatatgagagccacgacaatacctggtggtggcagttattactctattactcttattattactgtaataacccttgtaacttacagtgagccaagagtatggaatcactgatcatttcttattttccacatgctgaggagaagaatggttctcaggagagtggatagagatgtaggagggatgtggagcatctatggtttcacctctcttcattcgggctgttgacactggtacttctgtttccatcttggggattttttttttttctttcttccattatttttcttagtgaagtagaaggacgatgacaattgtgtgagatacgtggttcttagatcacctggagtttcttaagaaatgaacagaaattgatagatatatcttctctagggtagaaagaagaattaagggagtagcttcatcagaatgctggcttctttaacctctgggacactgatttttcaggcctttcagtggaggaactgggactccagcccctcttctgctggctccacacctatccattctcctgactctgtgattctcatttttgagggagtttaagggagaactctaggcaaataaatgattgccttccttctagcccagcattgtactgaatctcctccacactcagaccctgaagaactagactcagtaacctagaaatgccaaaaaagccttagtagtttcttctaagatctaaggttcagactcggcaaccaaccccaatatttatactgacttcttcctatattatttattaggttggtgcaaaagtaattgtggtttttgtcattaaaagtaatatcccagcagggctcagtggctcacacctgtaatcccagcactttgggaggctgaggcaggtggatcacctgaggtcaggagttctagaccagcctggccaacatgatgtaaccccatctctactaaaaatacaaaaaaattagcagggcgttgttgtggtgcatgcctatagtgccagctactcgggaggctgaaacaggagaatcgcttgaacccgtgaggcagaggtcacagtgagctgagatcgtgccactgcacgccagcctgggcgacagagtgagactccatctcaacaaaaacaacaataaaagaaaagtaatgtcccattgtatcctttgtattttccttcagtattgtattctctttcagtattgcttagatcagaattccatgaaattcctgtcggcacgtgattgtaggccacttagtagatctggggtgggtctaataatttgtaccatgttacctggtcatgctgatactgttggtcagatgaccagccactatttgagaaccattaatttaaactcatacaatccatgtgatccataaattttaatagcattgcgtaatgtattttgtatgagaatcttttttctggtaattaaagattttctctgttttagaaagttattttcagtgtaaattgcacccaaacaaatggatatgtatctagatttcaagaactagaaaagccctggattacactgtagatctgaacagctcattaccttacagttccactttgtgaaactaagatgatgctgttgaatgatcagttcttgctttaagatatagatctaaatagagtggccatgtacagccatgtcagtaataggtaagggcctcagaactaataactttcaactcttctccctgttttaattcatcttcaccatttgcttttggccttcgagtatattttggtaaagcagcatttattgctgtttgtaggaaccacttctaggagaagattcaagaattctgattaatataaacatagagagttaattagctggttaacagagcatccattctagaaagagctgtgagagatgaaaatgctattagataggagagagaaaaagagacagacaagcatgtcttcctttgtcctaaaacttcaaagaagttcctataaaagtggtcatttacatatagtatttcatttgggtggcttttgacagggtggattttcagaaaaattatggtgttcaaatgcaggaggggaaacttaagaccacgtggtggatactaacttcccttgattttcttctgcttttttccttccttgatatgtgatagagtaaaaataaactttacaaagtaagctgacttggttctacttcattgaatatagtaactacttaatgaatgtctattgaatcattttatactgaattagatttagagaaaaggtcttctgatagcatttaaaaagatttgatttgcacagatctttaagaaaaacattaggttctaaggaattttaaatatttcagaaacaaataatggaggaagcaatactgagggatctcaggtcagtcaacttttatgtcccacccactttcattcctagtacgacagtacttgcacagtatgggctttaatacatatgttttgaattaacgtaatccgaagttgcaaaagtcaatacagttgcctaatttattttgcaaaaatggaataaaacttttattacactatgcatttccagactttttatcagtgaaaagcaacttaattgacttgataaatattgttaaaaccttggggctaactaaattccttgactaccattttcaggccatgatgagaaacagataaaccgacttgacttttttttcactacaaagtcctcttagaactttttcacatgtataacattgaaaaggttttacaaatcacaaagagatggccacacttaaaaaggatagatggccatttagttatacattgagtgcagatttattgggtacctaatatgtgccaggcactgagctagcaatgttaagtgcagttcatggtttttttgtttgtgttgcttctagtctaataggggaaataataaagatgtaaacaaattaatatgatgcatatttccaaagctaaactgctgtaacagaagccaaaagaatgcagtgatagaaaataaggagtcttctcagacaatcagagtaatgcctcctgagaaagtggagagagctgatggaaggagagtattccaggcaaccaacacccaccccaaagtgggaaggactttacattttgaagaactgagaaagatcagtgggggctgagaagctgatggcatggagctagggtagagtgactgaggtgaccttagagagatgaacagagatgatatcatgcaaagccttgttcactgtccaaggtttggatttccttctgaggctttagatgggctttaacatgattggatttacttttagaaaatccacactctgggccaggtatggtggctttcgcctgtcatcccagcactttggaaagccaaagtgggcagatcaagaggtcaggagttcgagaccagcctgaccaacttggtgaaaccccgtctctactaaaaatacaaaaattagccaagcgtggtggtgtgtgcctgtaatcccagctactcgggagactgaggcaggagaatcacttgaagccaggaggcagaggttgcagtgagcccagatggcgccactgcactccagcctggaggacagagtgagactgtctaaaaaaaaaaaaggatcactctggttgctttgtggaaaaagaacaataaaaggggaagagaggagacaggcaggatcaattgggtgaatgttgcagtagctcagaggtgcattgatggctgcagagatggtgagaagtgggataattccaagtatatttgggaggtagaattgaatggggtgaagttgagtgatgggcggttctaaaaaacccagttttcttgcttgagcaactggtggatggcatttccttgatgcgaaagagtaagggatgaagaagttctttaggaaaatacattgtttagttgggggcatattgaatttgagaaacctgtgggtatatgagtggattcaaaagtcaaattgatgtttgaacatgtgagcatggagttgataggaaaggtcaatgctgggtattcagttgtgggagttaccttccaagagattatagtaaagccatggaaataaatgcagtggcttatcgactctccaaggaagaggaggagggaagaggagtctccaagaattctgagaagtcatgactaggaaaggataaaggataactagaaaaagtgatatcataggtccatcctttattggtgttggtgaattggatgtttccatgagttagttgggtatgtatacctgtggtcctgagtcactggacaattttagttgttgctaagtagatatatagtaataaatgactaaacttatactctcctttaacaatcttcttacatttgtggcatcagaccattggtagaggtgacagagtactcactgggaaccaggtgaatatctagtccttgacaagatcactttacctttttttatcactaaattgtgagtgggtcagtgatagggcttggacggtctttaaagtggcttccacttcagtgatggtgtgaaagagaaaattttgagccttatacatacattaaaatacagacttccattcttaaatcgttcttatttctagtgcagttggcagatctctgataattcataaagctggagtcttgcagaggatggacaagtgagaggcatagaaaaggatcagttttacaatttgtgtactagtgaagctttttttttttttagtaaaccatgaacaataattagaaatagacttaagacaagtaatatttgttttttaaaaaccaatgattaaaaattcaggccaccatcacttgaggtcaggagttcgagaccagcctggccatcatgatcaaaccccatctctactcacaatacaaaaattagctgagcatggtggcacgcacttgtaataccagctactgaggaggctgaggcaggagaatcacttgaagcccggaggcagaggttgcagtgagctgagattgtgccactgcactccagcctgggtgacagagtgagattctgtctcaaaaaaaaaaaaattcaagccaccatattatttgattttgtacaatacagaaagtacatatttttccccagtgaatataattgaattaccatttttattgaaagactttttttcttcaactataatcttaaagagaattttgaaatgcatcaagccatatacataattttcttaccttttaagaattatacctttcagctttttgtgatagagaatttgtggaaaagattttgtaaaatatttatttagaaacattttaaggaaaaaattgaaattatagaaaaatgcttcaagcttttgcaaatttattttggtaaagttcaaatgctttcccccctcataaaaaagatccatttatttcagttaagttttaagtatatcgctttgtaaataaaacttcaaatgaggcttgtttaccagatctttacaaatttaaagagcagaaatgtattctgatgtgtaatttgaatcagtttcctgttatgaagacagaaaagtctccattgtttccaatttttagaagcattagatgttacaagaagagataatgtaagaatgaaaagagaaattatttatgtactagattatatacaacttttcatatgaatacaaaaaagctcatttttcagaacatatgggattctgataatgttttgatatggatggtatagtttatccctctagacttgcttagtaataactttagtcttttaaaattacggtttaatggaaatcatggtaatatatatgtgatttcagctgaatacattatttaagctaggcttattttccatctagtccacataactttttaacagaaatgtcaaataatacatagatacaagctttattcacatattgtatacaatcagtgcttatgttgattacttctttcagctgaatagggaataaggcctcaaaaggtttatatccagtatttgagtacttttgttattctctttaaaaagtcagtattaggcactactggttactaccagctgaagccttacacagctgtgtatttagcatttaatcatgctaagaattgctaattagaaaatcaaaccggacaaagcatacccagtggagttgatacaataccatttctgtttgagaaccataaataaataatctttacgcattagtgtttcattataagcatttgtgctgaatgtggcaatatttaacaaaatgttttaactcactagaaataatttcttgatattatcctttcacagaaatccgtaatctctttaaaatatagccagccttatcaaaattaagtttctatttagcctttgatttctctttttttactttcttctattctgctccatttcagcattctgctgccccctctcccttcccccaaacttcccgctgccttctccactctgctttgttttaccctacattggaaccctgtggccacaaaccaactgtagcatcctcagttaaccttattgtggctcaggctccaaaattccctattcccttctctctctctgtgtttttattttcttaaatttaaaccgctttgtttctaaacctcagatacacttagctgcagcaaagaatgagggaaaagacattcattcaacactatgtgttaatggctgatagcaatttaacatattacctttcaagcagtagtgaatattttatactgaaattggaggtctagtaacagtgaggcattagtcaaaagaatcaataccagcagcataatctggttagtaaaagtcagagaggtaatggttccagaggattaggaggacacaatatgaatgcccctaataccagttttatggtccactcctacgggcgattatggctcaaactttgaggaaggaggtaaggcagcattttcatctgcatctcacatctcacggtctttgtgagttctacaatgctacagtgcctggcatggtgcttaacatcctcctgtaggtttaattatttcttttctgatttgagaataaaataggccggacacatcccatgttgctgtttagactgtacatattttgttgagtatgtgttcttgtttagaaatatacattttaggaagtaatgaagttgcgatttcctgaaattcagtaagtacacacttagttttaaatgagctgcatttttaagagaacatttaatggaaaaccaaagatctagagttttggtgtcatttcttctactaactccagtaataaacagactttttctggaggtctcatttacctgaacgacaccaagagctagaaagaaagtcacaaagacatttgagaggccaaaataaatgccaaaatgtccaggaactaacatttatttacttgactcacagtagctgcccttaggccttcatcacgcagagttaatttattccaattatatacctgctaaacagcttggttattttatttccaagcctatgaaggttaaaaacagcaagtacatttttgaggcaggcatgctgaaagcaatgaatactgacaatttaataacctgacagaacagagagatccagaactacttcatcatgataggcccactttattcatttgcaaaataaagagtttgggctaaacgaaccttcagaattacaggctaaaatacgtaacctcatacttgttttctaccagattaatatattttaaacctctggcagatttttttgaaattaactttaccatagaatacatatatgatatacatttagaatgacatgtggtgcttgttttatttacttaaaacagcaaaaaatacccttttatcattatgatcagaccggaaaatgacacttaaaaatagtaaatcatgtattcatttaaatccagtgactgtgttagctcctgagaagacaagatttagcagaacacagttgatttttgccctcattgaactacgaatcccattattcaacatttagaagtgctatgaaggaaagcatagggtgctgaagagtatgacattagggcctgggagtaaggaacagggtcattatgagctttttacatgagggttccaagggtgttccactgtagtttttccatccctgacttttggatctgtgctaagaaaatgtttactaggtaactgacatcaagaccctctggagagcccagtaactaaagctcattaacagacgaggcaaattttaggagcattcatctgtcctccctccatctgttttccttgctcatttcatttctttccatagtattttattgaaggtcaccacgtgtgagacactgtacactgtcacttttaaactcatctcctgtgacagagagcaaggagctccttcctcctaacatgactgacattttaggtcattctgatctttggttatgctgaatgttctctactttattggaaagtttaattcctcccactggctacttgtttgggttatgaattctctacatcattttgtgattccactaagttttgtaggtctgttgtggcccatttatactcaggcctgactggtatttttacatatctcttactgcagaagattttctagcttccattccaagctcactgaggatttctcacagactttcctaatatggtggggatcttagtagagaatatttatccttgtaaaagaaaatgcccagcccttcatacctatatcgttggcttattctattacttattggaaaatatttattgagtacctgtcaactgcaagagactccattagatgctggagatacaaaataaaatgccgtaaaccttaaagccctcaaagatctttcaggcaatctataagttttctagctcactgtgattccaatgtcctttccatttgtgaaagaacacccaaatggaaataaagaatagcagtctctgactctcttccacactcattatcagactccattcactcagtcattcatcaattctctcagcaaatatatattcagtatcaggacctattccagtcagatactcgaagaacctgccactacaagcctcatcttctaggtgttctgatgtccctggttctcttgtttaacataagaacattcacattctcattaaacctaggtgtagttgaagccaagagttggaatgggattatgtatccagaaagtggtgccatgaaaggtagccttactggcctttagttaatttgtaatgaagaatctgtgttttgtaatctttcccattactttgctttgccttttcttcttttattgtctcttgacttttccataacaactgagcatggtgccttttggaaaccatctttgagatgacctaaggaggttggttggtactagaatgagcacaggttttaacacaaggcaaacctgtgttgtaatcctgggtttactattactagttttaagtcattgggaaaatgatttaatttctcagaacttcaacttatccatgaaatgtaaaacaataaacaaaataaattgtgttaagtacttggcacacagtaaacctacttctccttagttgcctagtgttgtcttcctgaaacagagcttgcctggaggagaaggggatcatatgaaagcaatgaactggaatcaggatgatggatgccttattgggtgcagggaacatcaattgttgacttcagtttagtgtcatatttagtgcattttcctttttactgttaagatcttatagattgatagtttcatgtaaaaatatgtttgtttgtttttttttttttttgagacggagtctcgctctgtcgcccaggctggagtgcagtggcgcgatctcggctcactgcaagctccgcctcccgggttcacgccattctcctgcctcagcctcccgagtagctgggactacaggcgcccgccaccacgcctggctaattttttgtatttttagtagagacggggtttcaccgtgttagccaggatggtctcgatctcctgaccttgtgatccgcccgcctcggcctcccaaagtgctgggattacaggcgtgagccaccgcgcccggccaaaaatatgttttttagaagaaaaaagtttctcaggtttctacttctattatattttccaggaggaatacatttataggtattgactcaagtaggccctagctgacatccaaaataaaataagagatttttttaagtgttaaagttaaaaaatatgtatgatataccctaaggtagctggattttatttaattcaaagacatatgctaggagatctcaccaaaggacctgtattagttcgttttcacactgctgataaagacatacctgagactaggctgtttacaaaggaaagtggtttaatggagagcccacagttccatttggctggggaaatgtggaaacttccaccatggtggaaggcaaagaagggcaagtcacatcttacatgaatggtggcaggcaaagagagagattgtgcagaaaaattcctgttttaaaaatcatcagatcttgtgagacttattcactatcatgagaacagcacgggaaagacttgcccccatgattcaattacctcccaccgggtccttctcataacacatgagaattcaaggtgagatttgggtggggacacagccaaaccatatcaggatctatcttagaaaatatcaccaaaaggacaggctagtcttaccttatgtgaatctctgatctttgtggcattttagtcattgttatcggtcatagagtatttctgtggagaagttctactaaacttttgcatgtgctgtgttcaaaaaaagctggcaggcaatatgtaaatgtaatagttaaaattaatagccttaagaaaagctaaagctaaagcctgaattaataatttgtaatgaatctttatcaactgataatcaattgctgctaaaagaaccacaaaagctctactattggtggcattactatcttcatagacaaggttaccctaaaataagagcatcattaggagcttattccttccctttcatccgtgggagaaatctgttcctctttgttcagtctcactttgtttttattcccacaatcaaagcaatacttggaattttgattatattaaatttgagtttggtaactgccctggatgacccaatcatagactccaattcacggaagctatgagagagttatttcataatttaaaatgttagacctagaaaattttcataatacgttagttttttaaaaaactgtggcgtctgtaaaccctaatggatgctggatgctagacacaggtttattcatatacgtttatctggccagggttacagtgatatgaagacctctaatctattgatgatatttattgattcataaagcgagagattaaccattgtagtaaagtgactgtagtaacccatgtagtaaaccactgtagtaaactggagaaaaacgagagaggagaatggaacagaaaaaaaatttattagatttttggaacctgaaacagaaacaaacttgaataaattataagatcaaaatttctttattgcctgaattaatcttctcattttcttttacactttgacagaaaaaggaaaagttggtagacattatatttttcgatatagctgtgtactgaaaataaaatcaacgtgactgatagtttcaaaagtgaatttgagatgttacaagatgacatgcaatagtttataagttggaaatttacattaaagggatataaataaatatcaataaaaagaggaaagggggcttattatccttgtaaagtagttgagatgggaattagtgctacctagatgcttaacagcctcctcttgttaaaattgttaacaggacccttatgtatgtaatagaattgtaaggtcagatgcagcaacgtgtagctgaaagatgatgagctttttcaacgtatattaacctttgttgactttttttttttagcgatttatatctttgagatagtgggactttctgagtcttctgttctcatttttaagggaaacgatctattttatagtgttgttttgcagtttaaatgggataataaagtgagaaagcaccattttctgccatgctcagcacatattaggccctcaatgagcagtaggtattacttagcttgtagcaagattaacatatgattacaatttttgggggtagagttttattgatgtgttcttccaatatgagactgctcagctaaacctgatattttttaccagctaacttctcaggctgtgactattttgcttcctgaatcctcctatattttcacttgaatgagcagctgtatattgaatcacccagcatggacagctgaataaactagccctcatcactgcagtaaataaaagctcattttatttatttcatctttcttgtagctgttttagtttgtaagcaataggatttgttcgcttgtcatttggctttcttttggtgtatgagaaaaatgtatttcaaaaaaattgttgttttaaaggcccttaaggggaaagtgatagaaaataaatagggtggaattgtttaatgacaatattttagaaaaattctttttaatgcagaatatggtatttttattttgtgaattattatctgtgggtctctgagatcaactatgtgatctctgattagtatcatacctcaatcagaacaaaattagaaacaactactcctttaaaggattatttttgtccacaatgggacatagcttttttagatatttgaaagaagaacaaaggcttttttggttcttattattttaatgttgttttagtttgtataattgtaggtgaaggtccaaggtaaaaactatgaaacagtagtgcccaggacttaagatgcacagtcacatactctctgacttttttgtttgtattaagttataaaaacaatgtctggatgcgggtcaatggcagtggcttctgggtaattaggcagtcatattcaggagaacagaaagaaatactataaacagaagtttaaattttaatagttacacaggtttggagaatgatagtgcacctaaataagccacttgaattacagttgggactaataattaggcaggactgtcctttaaaaaaatagcaccgagccatatagtaaccagaagaagttgttcttgttttgtgcttttccatttggtactgataaagagaaacttatggggattagaaaaaatgttatattatcacatttttctgagtgaagctaatactagttaacctttaaatagcttcagggcattgttttagatagtatttcacaaacaaaagataaatcactccaactgtatttccttctgatagtgctgagcacagtatgtatttggcattatgcacagtaggtactcagtgaatctgttggacaaataaatgcatttgtagtttttacatcagtttctcaggtggtggaaaaactaagacactaagcatattacataagagttagagaaagggaatcactttggctaacataggcatttttttttttaatatgctatttggatcccttaaaagccacaacacatcaaacatgaaatacacatttctcaaactctcaatgcttctttctttctggtttcaagaaatactggtggttcctccttagaaatgtcatctatatttttctgttccattttatttctactcccattttctgcaaattgctgtgacctcgcgtgtgaacaattgcagcgcctactaccctgttttccaggctttacccttcagccatggtgcctttcttctctgaatctaatctacactgaaaacagtgactgaataatctgcaaataacacagcacttgttatgccatttctctcttgagaaatagttcttttggggccccatgtgtaaatgatgataaacacagcctgaattccctctcaaagtttccttatatttttcaaaccttgaagatggttaggaagtctgtctgtgaattgcatgtgtagagtgctataattaattatagcagaagaagctgaaagtaggtttaaggagctaataaccagattaggaatatctgatgctggcagtcagacctacctgttcattggtatccttctcattttatgcctcacagttattcacttcaggtaaactgatctgtttcccatttttaacatcacttcatttggaaggcttcctggaccctttgatgtttttatctgaatcccataacctattttagcatatcacattgaaatgcaatgattcttttactcacctttccctgcttggactgtgatgagttcttggcccctcatttggacctcttgaggtaggcactcattgtctccctgaggctggtatattatagtcctttcataatcataaactgaatggatgaattgatacaatttataatttgtgatctatgcctttcaagccttttgctgcctaaaatgttctatcccttgctttatgcctattaaaatcacacctatccttcctctctttcagttaatgcttattgagtgcctcatatctgcagggtgtgttgagcatggagttgtcaacatacatctctgcatggtccctctacagctgaaagtggcccacttgcctcttaagttatcattcttaggcactactttcacatgtagttatacattcaaatctttatgtcttaatattcctaatctggttattagctccttaaagctactttcagcttcttctactataattaattctgctatattcttctactataattaattataacactctacacatgcagttcacagacagacttcctaaccatcttcaaggtttggaaaatataaggaaactttgagggggaattcaggctgtgtttatgttgaagaacattcaatgagcaaaaaaattaacaaatccaaatattggttaaaagttgttagcaagccatgggaacgtgaatgaggataagcatcaagagtttcactaccaagttctctttaaaacaatcccagtggtgattggttggtgagtgcttaccatgaagaagtgtagtgttgagttctttacatgtactatttcattttatcctcatgatatcctatgaggtgtaagaagtattgacaaccccattttccttatcaggtaagagaagatgagtaatatcattcaagtcgcatagcgagatatcaagctcaggtctttttgaatgcctgtatttctaaccactgtttttggacactatagagttaattttttttcatcacgccatattacacataatatttttttgtgcttctatatcacattgttagaaaaataccacaaatggtaactgtgtactaacatttctaatattttatacaagatgaaaagagaaatagagacaagaaggaaaattctcttatggtcatcatagaaaaacctgcttatactaaagaagtagtcatcgaatatataccaatgaccttaagttgacatgtcatctgggaaaagacaatttcacaaaggtagatttgttagatttgtgccttgatatgatacacatgtatggcttctatttatctgagttgtatagggatagattagtgaaataggtagattttacacatttcaggactctgttgatttagcaaatgtttactgagtgcatactgtgagatagagcttgtctaggttgaagggacagaagagagaatgaaacaataatgtacatttttaagcaggaagtcagatgtaagcaattaaatagataactgcacagagacggaatatctttttccatattatgtagtatatgtaataagaagtattgcagagtatctatttattgatctttcaaagtgaattagctcaggagatatacttagatatactgttttgcaagatttatgtctgatatgatacttaaagaagaacttccacaggattgattagtgacaaaataaaagtgcctttcagggaaaaaattctagtttgttttcattgccaattaaaagaaccccgaatcagatatctttatttgaacaaaagagcaacataaactatttgtttgaaattcaatgtgaaaaaagctgctaatttaaggtatatcagatgaacattatatatatatatctgtatatacatacatatatctatatctatatctatatatatatgcataataaaacacttcagccttaatgtcatagaaacaatgtgataaacagtgaagttgtcatcattatgataataatcatcaagagtatcatgggcataatttctgttttaatgaaaaaaattattttccaaaagtagcatttcactactggggtttcacaggagaattaagccctgcagaaagacacacagatagtaccatttccagatgcattcaagagaagttaattcattgtacacaatggacaccttggatagggcattagttctaattctctcacaaaaccagagatgagaaagcaaattggcaagtctcttgaaatagatttccatgctatgtgatgctaataattcatgattatgatgtagtgttttttgatatgcctagaaatgacaatattttttgtttcaatttggtcaaattgttgaggccactgccacgttcatgttggagtcatagtcctgcagaaatgcacttccacaatcactggggacaggcttttgtgaagtttcagagattgagacagagctaaatcttttggaattcagaaacatgactattgatctagggaaagaagcatgtttccgtcactcggatttagtctgaactcttcattctaaagcagtttgattctgtttgtagaagtatacacaactagaaacagattgacaatttcagtggtaaataatttattctttttagaaagtcatattgacacctgtagagattttataaaatatatcaattataactttaatttgtaagtagtctccagtagtattgcctgagatgttataaaagatgtcaactgcttccttcctgaggatctatagtaataatttgtgattttcttttatgtcattacttacaatgacagttaaataataacaaccaatgctcgttgaatgcttttatataccagttaccattctaaacaatttacatgaattagctcttttgtgtgtgtgtgtgtgtgtgtgtgtgtgtgtgtgtgtctcactctgtcacccaggctggagtgcagtggcgctatctcagctcactgcagcctcagtctcccaggttcaaacgattctcctgcctcagcctcctgagtagctgggactactcagctgccaccatgcccagctaatttttttgtatttttagtagaggcggggtttcaccacattggccagactggtctcgaactcttgatctcaaatgatcagtccacctcagtctcccaaagtgttgggattacaggcatgagccaccagaattagctctttcaagcctcataatatccctagaaggtaaggactgcttgtatctccattttcagattaggagcatgaggtccaaggaggctaagtgactctagggtactggaatttgcaaagattacacagccagtgaggggcagaagacagaatttgaactcaggctgctggctcttaggcatcaccttgcctctgtcccttatatcctcttattgctttgtccttgttcttgacggttaattgacataactgtggaagaaattttgtgaacatagatagatattccaattcatggacaatgtcatgttcttgcttatttttatgtttagtggatgtcagttcggtgcactgtttgccagagagattttcttatttcctgaagactctaaaatccacttaattcagcctgccttctgaggtcctttgcctagttgacttttcatatataataaaagattccttgttttgattccctttatttctcttcattgtataggatagaatgccattccaacatatttcagcttactcagagcagatcagtatgtgataacatttatgtgctttattaatactcaaaagcatatgagaaatgagcagtatgcacttcttgcctgtggtgaggaaggaggggttgtaaatgctgtgagcatgagcatgtatgttcagtagtatcattaatatgtgatctcagacacacagaaaatctggtttttttttttttttttttttagtcaaatcggattcaggatacttaatgaatggtatttaggctgtattgtaatagttttgggaaaggcattattttttaaatcttgccattatggcacaaaaatgagacttcaggtatatataatttatttcaattttgtcatggattataattaaataagaatatatttatgaggaacaagctgttgacatgtttttaaaacttcagttgcagagcttagggtagattaatgcctatgcaataaaacaaattcttttaaaggaaagaaaagaatgaccagcaactacaaagtgtttaccagttgcgaaattggttaagatttctttatgtatatcattgtttgtcccttcaaatatatggcataagggaagaaaaagaaatgtaactttggggaatataatataaagtaatttcttaccattgagcaaatttgtaaaaacatatgaattgcttcaatttattaactttatccttctgaggaactttaaatagcctagattatttcacagagtataataaggccatgctaatattttaggatggagggcactggactagaacatagaactggagcttaattctaactctgcttctgattacctcctagcagttaatatctttcttcagtttcttcagctggaaaataaattactaacgcaatatgattttagcttttctttaaaattaacgatgctggggataatattggatagcatattggatatgtaatttctgatccctagggtactagaggttgccaatgtagtgtgggtagagtattctagttttaaagcaactcaaatgacacagagattagtattatactaataatttacattgcagtccttctcaaacctgcacaccacagaggaatcagtttgcctatttgagtgatactggcctagccatatttacagtcaatcagaagcgtgaacatttattgatttatttgaagtctcctgttttgtattcttctttgtggttgcgtcaattaagattatgttttaacacacataattgaaaaaaattaagtagctatacacagtggaagtttatttttgtgtcacataaaggaagttctgagataagcagtccagggtggtatgacaatgctgagaatcagtagggacccaagctgcttcaacactctgctctaccatcctcctgtgcaaccctcaaccccacggtcaagatggctgcttggctgctgcattctggccatcaaatggtgcatttttgttacatctcattgaccagaacattggctagctatgtgtccacacttacgttcagctaagactagaaaatgtagtctttagctgggctgcagtatgcccggctaaaagttggaagttgttactaaggaagtggaggaagtgtcttccacaatgatctacctatgtttgttttcttattttaaaaaaaaacccttaaactttatgaattaaaattaaaatttcatcttatgtcttttatagtattaactccttggtacacttttgtgttttttcactttgagaagtactgatttttatgtgattatttaaattcaataaacactgatataaaattatatgtgagctgctaattaaaagcagcaatgttttggatcagtgggttttttaaccactttcattggtatgcagagattttacccaccctgagctcacatggcgattctgcaattgccctgaggacttgaagtgtattaggatcattgattctcctctcttcaggtgctaaatcttttggggtgactccagctgtgtagtcacatttgttgcctttggagttgcattatttcagaatgcctggcaattggcttgccttggagaccttttccaagcatcttatctgcatgttatcttcctggaaccttttgcaaatagcacttattaaagaatttttccacatttgtatctatttaacccatttatgccggaggttgcaattttttgaatttttgcatgattggaaaatcagaacttggtgatgacttgagcagtaggatataaataactcccacatgcatagcattccaataatggaacactagccataagtgggtgtgagctattttttaaagcctcatatcttttgaagcagtctattactgcaactaacaaatatattaaagttgatttgtcaatttttatttaaagtataatatatgtattcttatattttatgagatacttagtccaatatcatgactacgatttcccattccttagaaagaattgttttcctggggatgtttctgacttttggtcattggtttttaatctattttgtggcatattcagtttgtcacaatcagtcttcaggttacaggaatccagaagaactcataaattcagggctttgtttaaaaacaacaacaacaaaacaaaacaaaaacaaaacttttgcgcctactctttcactgatatatttctttcttgctttttcatacaaaggttttgattctgcagatatgcaagtttttttctatcctgcaacaccttttttttttcatagaacatgtcatttccgttgcccaaaacatcctttttcatcctgccatttcctgtctctgatatagactttcctacctgaaactcaccttttcagaaactccttacttgattgatcctggaaagatcttatctctactttacttaacattccttctgtacttgtgttctccaattgcctaatcttagactcaggtttttagaacttgacaagatatttgagacctttgccagcatagtttttccttgtagctgttaacttagcggggaaaaattacttcctcatttttttcaattttcattctattgagtagtgtctcttaccaattttcctgtgaagttacatagtaaaataaagtacaccaagaaaatatgcagtttgacttgaaaagacttgacaagttacgattggctctttccatttttccacaattgggaatacttcaagtgttcttttctagtaagcattacttaagcttttttctttatacatgtttctcttttataaatgtagaagtctcacatgtcattttaattttatgtgaaatttaaggcaatttcaagattaaaagcaagaacaaactagttttccatatatacaccacttctgccttcttgctgaaatacactgataagggttttcctcctgccctctctgttacaaacatatcttagattcataagctctttaacatgctcactgttaagcatatgcagagaatctgtcattctctgacacccaggattagaagtagagaatattaatttgtggtacccaggaccttaagttatcttccagaagtcttttgaagtaatcattaatccaaaatatacctgaaatactgaagtgtaactttatcctaaattatcatgtataacaataacattttgggaaaatgtgcatagatttctgaaaagatttacaaatgagttattggaataaactcttatgagttgatggattttttatggatttgatttagcaaacaatgaaaattataagctatcagatgactattgagtgtacacaaattatggggaatacactatttgggatgccttgaaattaaaggaatttatagtctgcaaaaaaaaaatgacatatgtatacaaataattttatcacacgttcaaatatgaacagaaccaaagaagctataaagtactctcaaagaagataaattcttaaatttggcataattagacatgaattgatatagtaagtgacatttcaactgacctggaaggatctgttgaagttagcatttgagctgagcttgaaggacctgttgaatttcaatagatggaagtacttctaacaaaggaaatcagagagagtaaagtcaccagagtggtcagggatgggataagctaagggaatgtagaaccatgtagtgttgatcaaaggaggaagtaagaaacagaaggaccttggatgtcagctggtagttggaccaatgaaaatttcaagatttttctcatgggtattttttttttttttaagtaactagtgtagagaacttgagcattggcattgagtggagagtattttaataggtcttttaaaataaactggttggcattgggaagtgcacttttatgatgggtctaggagttaagataaaaagaaattggtgagaaagtacattttgggctgcttattcaaagacatacctctattacagacttctctgtgagcatagtgataaattgtattaatggaaaaaagtcatggtattgaaggattagaagagcacataaatccaaattttagttccacagaattggctgtatagaatataatgagatgaaagagtgctcttggcaggtcagttcctttaggggaggctgagggtcatagcaaccccaaatagctatgtttgataactgatgtttattctaacgttggagtctttgctgggtccagttaggatttttatcttattctgatctcattgtttatgcaggaaaagaataagatatatttttaaattgtttttatgtaaggtagtacatggaagagtacacagtctagaaggcactgtatcatggctctacatgtttctgcccaaggtacaaaatctttccttgagatgaccaagccactcatcccaggattaatgtaccattgcccataccgttctggatcgttgactttgttgcaaacgagtttacttcctgaatagttgtagaaatagattatgaaaagtggggagtgagatgaaggagaaagggtgatcaagttcctagttttctagtctatataatcacttaccccataaaagttaaagacttctcttcccttgaacatatatgctattcatgctcataagatagaaacactagagctaatgaaaatatccatgacgttatagtcgtagaatatgaccttattgcatattgtggcctttgcctagctttatacatactacactaggcatttaagagaagctgactcaagtatactttgatattgtcattgacctggaaggatctatttgagtgatttaccctggaaattatgtgaatttgacctgttttagccaagtcctgcacttactgtctttctctatatagatgtataatctagaaatgctaaatatcagtattacattagaaaaagagaaattttctttaagaagggattctttagttgccaatgaatttttgacatataatttaactgattataaatgtatttctaattggtttggaaatgttggtgtgcaacctttaattgcctgtcactaaactgttcctttagaaattcaactctgaaatcaagagaaaactgggctacaatttacagagatttaatataagtgcatttttggaaaatttattatttatttttaggctctttatttccccagtcttcagggaggaagtagggcagaggcagtattaatgtgctgttaatgaagctcatgaatctgaaatggactatgaacttctgaggaggaaaccatatcttgctctcttatattcctgacacctggtgcctggcacatagaaggtgaccagcaaaagtttgttaactgatattgaattattgatgaaatgaatatgcatgcaggttaaacaagatctgcactgcgctctgtctttgttggtaatatcagtggacttcaaaagggaatatagctaccagaattattttggaaattaatttggaaatgtagtaagtattacattttctttgctggagtattaatgaagaccataggttaatggattagaagtaggttatttggtattattggcctcaactttatccactctcgtattttcttagaagagataacttaatgtgtttaaagtcacaaagtaggtattcagtgactgttggttatgttctattctccctgatctttatgagaaaaaaaaaatgttagggacctcatgtggatctcttagtgctgtttttcagattccatttatgactcttgagaaagaaaccaaatgaagatgcattagagacatttcagcccctagagctgcaaaatctaccctagtaacgtttaagcaaccacctattatacctatagttgaggaattcagacagaatagcaggaacaacttttctgtgctctatactgtctggggaatcagctagaacacttgagagctagaggctggaatcatcctcaggcttgttcagtctcatgtttgacagttaaaattagctgttggctgagactttagttgagctagtagctacaacaccttcccttgtcttcatgttgccttctttactgatatggcatagtgtttggaaaagaagggtgcattttgcaagagagagagaagtaggtgtcaagtgtatcttttgttatctaaccttagaactcacataggattacttcttctgtaatcagttgaccagagaagtcacgagtcagccaaagcttacctgcccaagtttatacagtgtggacgtagcacctcttgatggggactttctgaaaacacatgtgggactggaaatactaatttagctgtttatgggaacatacagtctgccacacaatataattcctatgtcttttgcaatggctttataattttcaagtatgactgataacttatatttccctacattgtttttacaaaatagaccacttaccaattcccggtacctagttttttgttttttgtttttttttttgtaaagtaatttgcagcttattatgttatttagatgctgaaattgatggagggaagtttaaatttaaaaataaaaatcgattatctagatttttccacaataaacttttatttatttagtttgcatcatccagaatcctgggatatttgtttttgtttgttttgtgtgttttttctctaaaacagtttatttgggaatagcaagggtctgcaatgctggatatgcatgccattgcagaccatggatgcatctgtgaggggtttggagtaaggggaagcttttagagacaaaaagaagtccacataagttgttttgaaacaaagattattggttacaggggcttattctaggtggtggtgtttgttacttggtggtaatgcttgttgatagtaaaccatgtttctcatgtggaattgttaaattgaaagctgtctttttttatttaatttttcttttgtaatataacaatccccaactacattatttttaaaacaatattaagtctgcaggaaatttgcaaactcagttcaaagttattttttttaccagaaccatctgacaataagatttctatatgataccctgtcaccctccaaaacattgatatatattttgtgcacatgagggcatttttctgcataatcacaatacaaaccataaaaataaggaaattaacaatgatatattactaccatctaagttttacacctcaatgaagttttgtgagagccactaataatgtccttaataaggaaaggatccagttcagaattatcagtggcctttatttgctatgtctttaggctccttcttgaacacttactcagtgtttcttagattctcattgttttgatgttgttgaaggatatcggcctgttgtatagaatgtccctcaatttgggtttatcatttgttcctcataattggattcaggttttgcatccttacaggaatatcacagaagggatgctatattctgcatgttgcatctgattaggtggtacgtgattttgacttgcttcattattgatgatgtccactttaatcgtttgattaaggtgttacttacaagacttctttgctgtcacattactaattttacttggtagtcagaattggaagctatgtaaatatttctcatcagtctctgtgtctttatggcataatactgattatcatgaaaaaaattgagtgttttctttttgtttttgtttttttttctggaaagaaaggaggcagacagattagctagcaagactgcctttcttttgtttatgtaggtcacataatttagtagctaagcttgatttttgaaaggagacatttctttaaagtgctcaataatttgtttaaagttctagggaaacgacagtgttatttatcctgttaactgaatggcaaaataaagcagtgtacttgctgtttatcctttcaaagacttagattactattagctttcttgatttattaaaagaaataagtattgagcacctactgcatcttacacctaggagaagaaaagtcttgtgaataaactcacatgctacaagaagtgtggtaggtgccctgttgaaagaacaggtctcacaggggagaacaatagaggagatactttgttgtgatcttggtaaataactgtgacctgagggggaagtttcaggcacccaaggcaggctgtatttgggggagtgaagagtagataaaatattggtacctgatgaatctgaggccaggtttcaatactttatctgctcttcatttccccatatctacttactgtaggtacggcctcattaaaaaatataaactctctgaagacagaacattttgtttatttattctttgatatgtcccaagtgtcagatatggtacatagcagctggtcatggctatcaaataatcatttatcaaatagtgacccagaaattaggtgggtttccaagtccattaatcaaatttcttttgtaacgtaagaaagatttagatatcatttccgtagtgattttttttttctggtgagagtttcacctccgtttattatttttgtcctttttttctatctcgtggttactttccatatctcctcagtaccttgccatcatcatatcctcgggatgtccctgctgcttgtgttcagttccttgaaggtcttaagaaccttgaaaatttaacttttcaaagtcaaatcagggtttcaaattttgcttacttattttaattgtaactgtactggcaaaattaatcaagctcacaatgaagaaaaaccgatactgcagaatctcagtggaaatgaatacacccttctgggtgcttatttcattctcctgaactttcactgtgttgaaggcatcttttgagattttaaaaatagaaccattgccttgacattgatctctctattgcttctgtagcgtaattgtagtttatacccttctagatgatctgggaaatcatttgagttttctgaaaaactgaaaactagatttgatgctgcatgtgaacatttttggtactacttttcatttatgtattttaaacaactttattctgaaaagtccaaaacatagtgaacaaatacaactgagagaaaatatcttggtgcagaatgacctttttttttttccttttctcaatgtggatatcatttcagtccataatctgtgtattacttatcagatatcatggccagggaagagaacagcataatttttagttgacaaagcacttttatatatttaatctcatttaatctctgcagtgtgcttgtaaagtatcgtaagtgtttttagagatgaggaagctgggcctcagagagaataggtggcatcattaagatcatacagcaaattgtggaattggggtttgaagcaagcctcttgccaaacaaatcagtgaaaacaatgattggtgcatttttattttgaatggtgacctttatattttcagtgttgtttgttgttgttgtttaataagtcttggttaactatattagcagtagtcagagatcacatttgatatcccaagatttttttaagagcatttgctatcaaaatgttcactatcattttacctactaaattttgcagaatgaaattctttgcaacccacctgaccaaagcagagcattctttgtatcagaaatattaaatgggaaaagaggcctattgatgttggtgttgggaataagaaaaggaactccaacacccacccccctcatctcccattatcatctctgtgtaggattctctcacagtccaggcattcttttcctcagaatggatggggccaacaaaggatgcagtgttataggtttctctactgtgctggccccttctcaaggctcccattcttggaggagagaaaagagtgggtttgggttgcaggctggtatcaggagagatctggagtgcaaacatgacagcctagtgtgtccccacacctcagacctgttatcctctctagaggtctaaaagactctgatgtcctcagaatccaggatagcaaggatggaggtgggcttgcaccgttcaacttttaattatacttgcactgtttctgaagctcattttttaagaagctacttacaattttcttgcattgggatgtgttttacattggccacaatgaataaaaaaaaattgtttattttcggatagggggatgagtatatttttaagaaggcattacccaatgagtgtcttctttaaaagtttcaagatcttgctttccacttctttgaatattttttcaccatcttccattgtttgacatccctaatatcaaaacattacctgaaaataatgaaaattttatactttgggagtagttgctccccgagtctgactctggtacattgcttagcttctgttctgccccatctccagcctcacagagccaggctgctttaccggcttaagctggacagtaccacatggagggacatgggaggacaacaagcccctcactacattcttcctgtggtccagtcaaggcatttggtatataattactctaggataagaaatctggcaatactagaaacaaatcagtgtctatccggatcacgatcattaaaataaatgcaaatacttaacatatagcatctgattataggaaatagaatgtatattatccatatttccttattatgctaccttttcccataaaagacttcaaacagatgacttaatcctacaagaagataaaatgattatttttattgtaaggttgtcttttcaaaagacatagaaaattactttatagctataaacaaaattactttatagatatctgttacttaagttgcataggaatggaattattcattctgatatagtgaggggagtgcctatgagtgttgctgatttctggttcagtatttggtcccttattgtgatcattttcttttcaatttgaagatgtcagtttttcccctatacccatagaagtagtccgggattgggcatgtaagcaggttgagcccagatgtcgctccattcctgtcctgccatctagtggagaaatgtgcatgcagtgctggtctacgtacaagacgatgcaatttctaaattcctgtattgagtgaaatggaaggcttattctgtaccttatccacaaatattcataacttacttaagaagtagtagtactggtagtaaatggccattgatgagttaccaaaaaagatgggtccttaaaaatatgctaagtataagagtaacagaatccccaaaatgaaaagtaataaaatctaacattgcaaatataaaaatgtaaaataaaactctttggtattggcacagagatggatagatcattggaacagaatagaattcagaaacagactgtgagggtggcatttcaaataattgagatgatgagatattaaataactaatgttgacaagactggctaaccatttggttaaaaataaagatggatgtcactgttactctttccttcagaataaattctcattggataaaagattaaaacattaaagaaatgatgctgtaaaattatgaaaagaaaatatggaccatttcaaagataatcttgaagtgagaaaagcttgctaataacagtaaacccagaggccatttaaaaaaagacatttatccttccagcaaacaaacaaaaacagttataagaaaattacaaaaaaataatatctaaagggtaaattctaggttctattctttaaaatgaattaaatattaatgaaatattaaatatcgacagagtcgatatagacaatatgaaaacagactatatagacaatatgaaaacaatttgaatttgtttctctgattattcatgtgaaacaaaggttcttttcatgtttatgccattaagttgtcttctgtgaattgggtgctttctggttttctggtggtgtttgtggttttattccccctattttattttagtgttaatcctttattatgtgtattgtaatatttctgccagtctattaattattttgttgatttttaaaatgtctttttaaaattataattcagtttaacttttaggctgggcgtggtggcttgtgcttgtaatcacagcactttgggaggccaagacgggcagatcacgaggtcaggagatcaagaccatcctggctaacacggtgaaaccccatctctagtaaaaatacaaaaaattagccgggcgtagtgggggcacctgtagtcccagctactcgggaggctgagccaggagaaaggcgtgaacccaggaggtggagcctgcagtaagccgagatcgcaccactgcactccagcctgggtgactgagcgagactctgtctcaaaaaaaaaaaaaaaaaaaattataattcaatttaacttttaatcgctctttgacttctactagcggagggatagaacctcatatttttttcttcaatcagtagctgattgtctctgtcatcatgttccattgtccccatttattcagatttccttccttctttgtcctttagaaaagttttcatgttttcttcatgtatatttggtatatttggtatatttctgttaggtttatttgtaggtctttatgaattttgttgctattataaatgaattatttagtccagttttaaaatttggtatttgaccaggagcagaagatatttgaccaggagtagaagtacttttacttgtaaaaatgttacatttctggagttaggatttgtgtgtgtgtgcgtgtgtgtgtgttgaacacatttaccatggagtttgttttctaagagctgttattaaataaatttgctttttataactgggtcttaaattccaaaaaatcctgtatgtttatatatggctaagatatcctgagggcctcccaaaccactggacgatatcagtattcttatcgtgaagttccaatttcaaagttttgccgtgagttcagcaaatttaagattgcttcaacttctggctcttgcatctgttcatgactccagaaccacctgcttgtcaaccgaatccaaaatccaaccccttcaatgttctcataaagcatccatcacaccaaatgttctgtgaatttaggctgaagattagagatcatggggaggggttacattgagggacagtaaggcatccacttgctcactgtctctgctccagcctttcatctctaactcaggaaataggagtttgcatgtcaccttggttcccactcttccttctaagccaagtggaataatatcttctaaaagtactgagattttttcctgaaggaaacatgatgaatataattttttctactctttcacgtatcagtaaaggctatatatggtgcttacatacaccatgtgtattcatatgattttaccgtgtagcatttatgtttaagtacatctaacttaggactgtacataaaattttaaatcattctgctcttgtttatttcaatctacggataacatttaaattttcagcatcttacatatacttggtaaatgtagcagaatataaaagttttaattcaaaattgatatagtctctatttcttttatatacatatgttctttgacttacagtggggttctgtcgtgataaaactatcataagttgaaaatattttaagtcaaaatgtgtttaatacacctaacataccaacgtcatagcctagcctacctgaaacgtactcagaacacttccattagcctacacttggagaaaatcatctgccaagacagtacacagttgtgttttggccattcaacctcatgattacattgcagagtaagagctacagctcactgtcactgtcccaggcatgtgacaagccttggaaaagatcaaaatgcaaaatttgaagtacagtctctactgaaggagtatcgctttcacagcatcataaagttgaaaaatcataagtcaaggattatctgtatttataaatagagcttcctggaaaatacaatgttttggtaaggttttcttccctaccagataatggtagcctattttacttactcagtagctagaaggatgtacctcctttctgtcatcagtctcggtcatgcagtgacattattcgctaatttttgagagacaaaatgtggtctctctgtcccctgctgagtacaatagagaaagttaatacagatctctttaggtgataaaatgaatagaaaagggaaaaagggaaaggaaggaaaacttaggcttaatgttccattaaatacttaattaaggggtgcagtgatgccattgtgaccatgctttttttttttttttttttttttttttgagacagaatctcactctgtcgcccaggctggagtgcagtggcacagtcttggctcattgcaagctccgcctcccaggttctcctgcctcagcctctcgagtagctgggactacaggtgcccgccaccatgcccagctaatttttttttttttgtatttttagcagagacggggtttcaccatgttagccaggatagtctccatctcctgacctcatgatgcacctgccttggcctcccaaagtgctgggattacaggcgtgagccaccatgcctggccgtgatgatacttcttattgtgcagtactccttagctacaaatcacgttatgctacaaagtggtgccaaatgcagaagcatggctgacacaggcatggcaataactcttcctgagctagagacctgcagggtctatgagatataactgtggcagctcactctacacattatgaacacagaatgggtcaggcttctgctttcatgactgcattatggcataggagtcatcaatgcacagcaagtgtgtcattcttacagtggaattaatgtgttcctcaacgtgccgtggctctatttattttcctatgggaaactgaagctgggtgtctttggcaaagatttattcaaaaggatggcatcattaaaaacaagcttgtgcctatagaacaaaatgaagtaaggatggtatttcttaaaatgaactgctttgattttcaacacaaatcaatcatactggcaaaaatttgtaaatgatacattaacaaatttttgccagtatgattgatttttcatatgtttaatccacatcttttgtttgtgtctgcatacaaatttttttctgaacatgcatcagttgtcatttccaatttttgacctttttctgagattttaagcctttagcaactgattttttaagttgtttttgttacttacagatcttaccaaataaaccacatgtcctcatttcagttagcattatcagatgaaatgttgtaaacaaaagcagttatttagaagaaaatatcatatcctttactttctaattgtttaagaaaattacttaaaaggtttttttttaactgggctgttaataacaccaattataaactacattggtcttcgtaaaacttactgccatgttttgatttacaggatctccaaagatgggtaaatggtgctaatgaacatggctttgtcttggtgtcttttggagctggtgtcaagtatctgtcagaagacattgctaacaaactggcaggagctctggggagattgcctcaaaaagtgatttggaggtaaggtaataatgtagattgtttctttgctattgacaatcaatatctccttgtttagtgcacaggtcccagtaaagcacagcacattgtttccctgacaagattagcaagatgcccttgactttcattttgtttcttagcttgttgaaatctaggaattaattcataaggctctatgatggttaaagaaacctctgacctatatagcacagaaagaagatatgattcagaatgacttttccttgtgtcagatgcatacttacatttccctcagagttctaccctcgtttactcttttattatttattatgattttaaaaattagttttaattgcatgcctttttatatactccttcaaatcagttttgaaatgaggaagaaaatgatggattaacgaatacctaaaataccgtggactcttttgggctcccactttgtctcctttacattatgtttttgatttattttatttaagaaacctggcctttaaaaacacaatcacgtaccatttaacacggtttaagacagaaccatagattgaccccagcttcttttggaaggcattgccagcacatgactgtctttggaatttccagcccaatgctgaaaaatcagacgtgaacactttatttagcgtgtatttattgagcacgtactaccactgttgaactctagggatacaacgtcggtcccatagttactaccatgagtggaagaaagtgccccttaagccattgcaagtaggctttgagtaatagagattttccctttatagcaaatgagtaaggattagctcccacttctcctggctgaactatgcagtgatatttattttattctaactgttcaggacttttcccttcagattcgagtcccattgggtttcctctgttaggcttaaccccagaaagtacctcttctgcttcatttaggacagtttatgtctattccattcagactcttttgtcaccctcttagttgttaagcatatttctgttttatcttttaaagatcaggcaggaaacaacctaattatgtgcttcaccccacaaaacttttatttctggtgaagctaaagaagagaacttactgatttttttcaatacttctgccttccctcagactcagggtgttaaggatttagggatattgactgccatagcagtggcagctctccctgctccttcttgttccagcttctggctgtttgtggggaataacttctagtgtaggtttatttgtttgttgtttgtttgtttgtttgtttttcccatctctgtatgtgtataggcgtgaggaaccaatggaaaatagatctctatgtaagcaaattatttcttgtttttcctccaaccagtgaaagtttttattaaaaagaaacttaatcaaatatttgctgttaccaaagcatggtttcattcttaagaatatcaacaaaagatcatcaaacatttattttaaatctcataatttaatcagagagcccatactatgagtaaggtttgatttttaaaagactaattgtctggtgtacattttaggttttctggacccaaaccaaagaatctaggaaacaacactaaactcatagaatggttaccacaaaatgacctgcttggtaagtcaatgatgtgtggttacttacttggctgttaggttttaattacataaatgtgactttttttttttttttacttcagaggttcatacggtatacggtatgtatgtagtatatggtagagttattatgttttttatccagtatctcaaatcttaaatttgaggccaaaattttaagtctttatttattggaaaacagtttgtaaaatgtaaacctttgggcctctatattaaaatttttagaccagccatcaattttaattatctggaaattatgtacttaatgaactatataaattagtagtgaataagattatacctaattagagtaatcagatgaaagtagaacagttaaaacaataagaatgtagatttaggttacaggtttgttacagatggtctgagaaccaagagaaattagaagttattcatttgtctgaaaccaaagagaagcagaagaccatgggaacagtcaatttattttaactttaactggattatctgctctgtttagtcctaaatcattgggcatttttgaagcattttatattatttaatcttggggattttgattctcaaaattaaaatagtaattagtatatgcgtatcttttaagtgtgttttttaactaaattagttttttaactaaatttaactaaaaaccagtaaagaattttatttatgtatataatttattttcatctagcttattataatactattctataaatgctaaaactaaagaaaaaagaatacaaggcaatttacctttcttgatccttgtatttttttatttttaaatcttttatggctttactgttatgacttagattccttagaagataggaaagaagcaggaagtttaagtgagataacctgactatcaactatttcagtgcgacagtgtgacactgttatgtatgaacatctaaacttttattgtgtgtgggttttccatttcttattgtttttctttttttcttttttttgactgtgaggctctactgcaaggtccatgcctgaaaactctcctcaagtccatagctgctctaggcttctcagtgtgagaactctgactttttcaagattagtatcttttttaacaataggcactatccttgtgagtcctctaatagcttctaactatgatcaaaagattcttccgggatgagaagtaggaaccaaatcaatgtctttcccctcccctcgtagccgcccctcctctttacacagcagctctgctttatttaactgttgggtttggtggtaggttttgttcaaagagaggggtttttgctaaaaataaagtttgaaatccacttctagggcagatcctttagttggacctaagagtcagaaaagccacttgtgggtaagggctagagacactgactaaccaattccaccagtcttcagaatggaagagctctgggagcaccattgagaccatggttcccatacatattaattttgtacctggcacatgtgtattttaaaagatcgacatttcagctagctataatttctttctggccaataacatatatcctaagtacaatgtttttgttttgttttgtttttacaactcttatgccaacttttgatcccttttatagaaatgtaggccatttaccaggagagtaaatctaggttttgaacttccatattaattttgacaaattatcttttttattcccataacaactaaatgttatgtgatgtctcatgtcttacaaatgattataaatgtttacctctacatgtttgagcacataaatgtaaaattaaaccttaaaattgtgaaatattaatgctgatagaacttgaatgttgtgaatagtgattacaacatttctttttggagaagcacacaaactcttcatggacttctggaatccagcccttttttacattttttttaaaaagtgtttttgactttaatattgataaacatttgagtagccagaaagtagatgtctgttttttcactctggtattgtttggcatttcttgctttcattggcttcataataattattggccatttaaatatgtgttgttagtcatgcaatatttgtgttaaaaatagtaatatacatttcaactacttaaaaatggcttttaattgatatatcaaaatctgacaattaggtatataacaaatattttaattggtgtagagcaggaatcagtgaaattacacctttaggaatcctttatctgaaatgcatgtttactgtagtgccgatttttaatgaatttctgggaaaatctcttctgtagagtaataatgttgtaagttgttttctttttcatctttcttcagggcattcaaagattaaagccttcctgagccatggtggtttgaacagtatttttgaaactatatatcatggtgtgcctgtagtgggaattccactctttggagaccattatgatactatgaccagagtacaggcaaaaggcatggggatattgctagaatggaagacagttactgaaaaagagctctatgaagcactagtgaaggttatcaataatcccaggtaaggtttcaattaacattaaagctgatgaacttacataccacagtatattgtcagtagccaattattttcaatagattgtcaataaattatcaaattatggaaatatcctttagattcctgtgataatgctttgtgcatgttttctattatttagaaaatgaaaacagcagtcatttgaccagccatgttatgacaccagataatattctgcaaggatcttccaaacagggagaaactgcaatgggaacaatctttggatatctacattgtgtcaaatgttatgtgctttatttcattttcatacttataacagctgtatatcacagtttttattatccacattatagaggcaaggcacttgatattcatggaacttgagtaatttggcttacacagcaattgtagttgaaattagaagccaggactgtctgattcccaagacagtgttctttgtactgcatggtaagcctggtgttgctgggtttccctagcactgagtattgcagaaatacggagatttatttactcaggtgaatgatgaagcagaatctttattttgctttttaaattattgatgggtcctgagttaagctagttcaccaatgagtctcaaagggtgaagaactggcctgtgtagttttaaaacaaagcagcagttttcttcatttgtagatattatatttaatttaccttgcatttccaatagcattaaatattagaagcgtataagctttttctttttatgcctaggggatatggcttaacactgagaaacacttgagaaacactgccacattctaaggaacaaccaataataagaaaaattatttcatataaaaggatgcagcttgcatataaaatgctgaattcaactgaagttcattatgctgcctttatgtgagctcaggggtgaccttcatgctctggactcttaaaggatccagtgtcggatacagctctgccattggagcaatgtgttccataactagggttgcctaagtatatcccttcttctgttatctatagtttttctttaaaggtgtgcttttcaaaacatgatgttatttcatatacatatatatatatatatatatatatatgcacacatacatatacatcatgcatgtatcatatatgtgtgtgtatgtatgtatctatcttcaatctttcaggaaagtttgtaaaatatagccctaagtagaattatggggaaacagttgcagaactgctgaaattggctcagatgaaaaggaaagagcaaaaatctaggttattcacaggaagttagtccagctgtgttttgcgaggcatgaaccaggctgaatcagagcaagaacaggttgcaatcttaggtcacatggcaattaaattccagctatagaatattgaagacatgtaagtgcttaatttaaggattattcaatgcagtgaataaatttatatcattcccaaaagtatgcacatcagataatgagttaactgcatgtaacttgaaaaccttaaatatttaactgaaaggattttgtgcatagaaagatgtcttagtcaatgtaaaaatgccagtgatttgtgtagcatgtcctttgctaaaagtcattatataaactgaagtcacttatctttgtttccaatgtgataatattccacatttaacaggtgataattattgaaaatattagtttgcctcactaatattgtgtccgagatattctagtttaaaccaagtaactaatactgtaaaagaagtattccttttatgaagccagcattatcctgatactagaactgggaagagacacacacaaaaaagaaaacttcaggccaatatcgctgatgaacatcaatgtgaaaatcttcaataaaatactggcaaaccgaatccagcagcatgaggcgggtggatcacaaggtcaggagatcgagaccatcctggctaacatggtgaaaccccatctctactaaaaatacaaaaaattagccgggcatggtgatgggcacctgtagtcccagctactggggaggctgaggcaggagaatggcgtgaacctgggaggcggaacttacagtgagccgagattgcaccactgcactccagcctgggtgacagagcaagactctgtctcaaaaaaaaaaaaaaaaaaaaaaaaagcttatccactatgatcaagttggtttcatccctgggatgcaaggctggttcaacatatgtaaatctataaggtaatctatcacataaacagaaccaaagacaaaaaaacacatgattatctcaatagatgcagaaaagcctttgataaaattcagtatcccttcatgtaaaaaactcttaataaactaggtattgatggaacatatctcaaaacaataagaggtatttatgacaaacctacagccagtatcatactgaatgggcaaaggctggaagcattccctttggaaaccagcacaagacaaggatgccctctctcaccactcctattcaacatagtattgcaagttctggccagggcagtcaggcaagagaaagaaataaagggtattcaaataggaagagaggaagtcaaattgtctctgtttgcagatgacatggttttatatttagaaaaccgcattgtctcagccccaaaattgaactgaaaggaacttcagcaaagtctcaggatacaaaatcactgtgcaaaaatcgcaagcattcttttacaccaacaataggcaagcagagagccaaatcgtgaatgaagtcccattcagcaatcactacaaatagaataaaatacctaggaatacagctatcgggatgtgaaggacctcttcaaggagaactacaaaccactgctcaaggaaatgagaggacacaaacaaattgaaaacattccatcctcatggataggaaaaatgaatattgtgaaaatggctatactgcccaaagtaatttatagattgaatgctattcccatcaaactaccatttacattattcacagaattagagaatactattttaaatttcatatggaatcaaagaagaccccctatagccaagacaatcctaagcaaaaacaaccaaccaaaaacaaaaaaacaaagctggaggcattacgctacctgacttcaaactatactacaagattgcagtaactaaaatagcatggtactggtaccaaaacagacatatagaccaatggagcagaacagagacctcagaaattacaccacacatctacaaccatctgatcttctacaaacctgccaaaaacaagcaatggggaaaggatctcctattcagtaaatggtgctgagaaaactggctagccatatgcagaaaactgaaactggaccccttccttacactttatacaaaaattaactcaagatggattaaagacttaaatgtaaaactccaaaccataaaaaccctagaagaaaacctaagcaataccattcaggacataggcatgggcaaagacttcatgactaaaacaccaaaagcagttgcaacaaaagccaaaattgacaaatgggatttcattaaactaaagtttctgcacagcaaaagaaactatcatcagagtgaaaggcaacctacagaatgggagaaaatttttgcaatctacccatctgacaaaggtctaatatccagaatttacagggaacttaaacatatttacaagaagtaaacaaccccatcaaaaaatgggcaaaggatatgaacagacacttctcaaaagaagacacttatgtggccaacaaacatatgtaaaaaaggttaacatcactgatcatcagagaaatgcaaatcaaaaccacagtgagatatcatctcatgccagtcagaatggtgattattaaaaagtcaggaaacaataggtgctggtgaggctgtggagaaataggaacgctttatgctgttggtgggaatgtaaattagtttagccattgtggaagacagtatggctattcctcaaggatctagaaccagaagtaccatttgacccagcaatcccagtactgggtatatactcaaaggaatataaatcgttctgctataaagacacaagcacacgtatgtttattgcaatacaattataatagcaaacacatagaaccaacccaaatgcccatcagtgatagactggataaataaaatgtggtatatataccatggaatagtatatagcattaaaaaggaaagaggtaacgtgctttccagggacatggatgaagctggaagccatcatcctcagcacataacacaggaacagaaaaccaaatactgcgtgttctcactcataagtgggacttgaacaatgagaacgtatggacacagagagggggaagaacacacaccagggcctgttgggggtagagggtgaggggagggaacttagcggatgggtcaataggtacagcaaaccaccatggcacatgtatacctatgtaacaaacctgcacattctgcacatgtattccattttcttttagaagaaataacaagaacaacaaaaccccccaaaagtattccttttattaatccacaacttaagtaaaattacacatcttacgtctctgtttcctaatgctttggattcatttaataaaggcctattgcttttttgtttgtttgggaggattcctttgagtctggagcttttattattacaaaataagttagaaagaaagatggagaatcgatcattattaacttcgcacatatccaacctgtggtcaacttttaatagaagatatttatacttttgtaaaatttaatgtacatgtgagccccttacaaggtaattgttttattaaaaggggctttatctaagagatctcttggaataacttagaggtgtctggagtgaccatttttaatcacactatttttttgcaatattcatattcttactggaaggaattttgagttgtaaaataaactatgctcatgggacaatgccactacattaaatttgagaccagtttcagcatggaaaatacctgcccctcaaaaatttatctgtgagttctccaatattcctttccagttgatccatggacctcctctgaacagaatagtcatacaaaatgaaatcggttagttagcaatccagctttataagtctactcctaggtgggactaagagtctgaccgatgaaagtccctgttcagataagctgagtcagatgtcaagagcttttctgataattagtgatctaggaccaagtaaacatattggagttccatatgagttaataatttattcaagagtacaagaagtgagattttccattaaagcatctgtttaatctgtttaatcatcactagagaaagggttatatacacagtgacattaaggtacctgaagacttaagattgtttttatccttcttttccatctttgttaaaataaaagattggattttattttctaagatgtcacgtttcatttttgtattttaaagatactcctttgccccataagcattttctcataaaatggagtagtagaaactttctagtttcccttttgccatcagttagaaattatgataaattacaaagcaactgaggatggccttttaatatttggtgaggtttttgtacttttaatacaactagatttattatttggttgtaattttcttatgaggcattgatgagagagaaaacgtgcctgttaattacatacttttatgtaatagccttcatttgttttttctctcactcctaacaaccttctgttcactgcctctcaatttttttgcataattgttaaaacttaatgtttaggtctagagtgaaatcataaaaaataaaggctcatcaaatcaactcataaatatctgagtagatttttcactgggctttgtaatcttatagctccatcctcacatttctagtggctctctcgacctttcctttcattacatcccaaactgtaatcatttccagcagcatgtcccgtgttctgtgttactgtgtcctgttaattaactctgccatgtgagtcattcaagctggaaacattgcaattacatatgatctctccctttcccttcacatttaatccacacttttaccaactcctgccaactcttctactacaccatttcccttccctttatctgtctaatcccaccaccatttttttagtcagtctctcattggtcattattgaggtctttttaatggactttccatcacgagtatcttccctctgctttaacagcctgtctccctgatataatggctctttggttctaagaaagaagctattatatcttgtcattcagaatacccatggggaagactcatcttcttccaatctaatttctaactaaacttcatactttttccaaatgaatttgttctgggcatattctcagtctcccacttttatgatttagtttacactcttctcttgatttatcaagtcttcacacatgtccaatcttttgttcctctataatgcacaactcagtagtgctatatcctccatgatagattttgtatctcttgaggtggaaattatttcttatgtctaaacaatacaaacttcagtcatgaattcatgcaagggggatttagccatttgtcaaagattggcacatgaatgtgcagtcacatgtttttagattaaaataaaatgcttatattttatcactttgtgattccccattttccttggtcttttaatcatttaagagggtgttttctttatacatatatacatgcatacattacctatacatatatactgcatataacatcaaatctgacttcatggtgtttcccaactcttttttatctctttaataatatatcttcaccccatatttaatgttattttaaattaaaacaaaattaaatattattgcttaaaaagtgatagaatgaagttctgtatctttttctccatctttcttttagaatctaataaatttagtttccatcctggttgaaacttgttgatttatactatttaaaagtatgtggagagaagaactacatgtaatgtagtgtggaaacagcatagggtttggagtcagaaaattctgggtctcaactttgtaacataatcaagttagtctccgattttcatttttctcaccaatttaaaatacattttattgggttaacataagataatgtgtttaggccgggcgcggtggctcacgcctgtaatcccagcactttgggaggccgaggcaggcggatcacgaggtcaggagattgagaccatcccagctaaaacggtgaaaccccgtctctactaaaaatacaaaaaattagccgggcgtagtggcgggcgcctgtagtcccagctacttgggaggctgaggcaggagaatggcgtgaacccgggaggcggagcttgcagtgagccgagatcccgccactgcactccagcctgggcgacagagcgagactccgtctcaaaaaaaaaaaaaaaaaaaaaaaaaaagataatgtgtttaaagcacttaacacagtgcttgtacatgcaaggtacttactaaagaatagttgttttaattatttcccctttttaaatgaagatatgcataaatatagaactttattataagcatcatcattctgtgttttgtcccctctccatagctaccgtcagagggctcagaagctttcggaaattcacaaggatcaacctggtcaccctgtcaatcgaactatctattggatagattatattattcgtcacaatggagcccatcacctacgtgccgctgtccatcagatctccttttgtcagtattttttactggatattgcctttgtgcttttgcttggtgctgccttgttatactttctcttgtcttgggtgacaaaatttatctacagaaaaatcaaaagtctgtggtctagaaataagcatagcacagttaatggacattaccacaatggaatcctcaatggcaagtacaaaagaaatggccatattaaacatgaaaagaaagtgaaatgagccaacagcccaggtgatagaaataaattggttcactcattgaatttttattgctattatttagtctaacagctactaaaagtaaaacatcagtaaacaattctaacatgcccttatgagatctactaatgaaattctgtggaattaagatggctgtaaaaagcacaaacctaaaatgcagaaatgtattttattcaaatactgatgtagagagttttggcactgaaccttttagaagccttaattatttaaatcaattcagtgactgtgtcagaccttagttttaaatcttgatatgtgcgtgtcccggatcaggaatggtttcatttttcttaataatgtgtgtgtgtgtatgtgtgtgtgtgtgtgtgtgtgtttgtgtgtgtgtgtgtgtgtcctaattaagagaatttttactggctgcttgttacatttgttgagggtacaacacactcaagaataaagtaaaaggatagtcaggatccagatgtttcttttctagcatttaatgtgtgtgaactcagaacactaccatgaaagaacacttccccccaaaactggatgcagaggaagaaaaaaaaaaaagaaatggcacagttttttgtatttttttttttagttattttttgttgttgttgtttgtattgtttttcttttctgatagagtatggccacttctgggggaaaaacatgtaattaagtaaatgtatacattggttttcacgttttacttttgttttcccactaccaataattttcctctggaagaattttatagttttttctatttcattttaatgagtaacaatatgttaaatgcataattaagacaaagcaatgaaattctgactttattcaaagtactgaagattattgcttctagggcatttttaaacagcaccattgtattgttgaatgtttatgtaactgatggcttttctataatgtaatttttgaatgttcaggtgttacatttccaaagtttaacttttaaaaaaccatcttctgatcccttttattgtctgggccatacaatctatattacataggtgccaacatttaattcttttaaatggaacatttgcagttttccatattggtacctgctttttctggagaggtttgagatcttgttaacaaatcagactttacactatatacagatgtgacagataaattgaaccacttgtttgtgaaaatgagttcctgtcatcttcctcattcactcagccctcaccccagcagccttttccggtcattgtagctgacatggagcagtgacagtattcatttgagaacagggatgcaagtcacagacatcataaaatcagggtctccctgctgaagcattcactagttggcaactatgaatttattccatgtcattctgtttacttagcacttgcactacccttgttggttgagtgtatgctttatttgtttctagtttgaaatcccacatctgatagctgagagtaggcaaatacaacatttacctaatgtcattcactaacatggaagagttgtgaaaattctagagtgctgtaaatccttggcatacactatgacaaacaacttcattactctcccaccaggagctgctctcctgcacttagaaataatgtcacaagtagttttctaatgtacaatgcagacaaatgtactgctctctgaatacttgaagaaatggtattatacatacatagaaacttattagttataccttttcacaatcttattacgatgttgccgttaaaagggaaaaaagacacaggcaatgaatggtgggatagtaagaggacttagagtgtatgaatgagttgattttacttttttggaatttgattaagttgacagtaggcactgattggatgattaaacataagttaatctccactgtgataaaaacttaaataataaacatgatttaaaataga

SEQ ID NO: 2 - protein, 541 aa, synthetic construct
MKSYTPYFMLLWSAVGIAKAAKIIIVPPIMFESHMYIFKTLASALHERGHRTVFLLSEGRDIAPSNHYSLQRYPGIFNSTTSDAFLQSKMRNIFSGRLTAIELFDILDHYTKNCDMMVGNRALIQGLKKEKFDLLLVDPNDMCGFVIAHLLGVKYAVFSTGLWYPAEVGAPAPLAYVPEFNSLLTDHMNLLQRMKNTGVYLISRLGVSFLVLPKYERIMQKYNLLPEKSMYDLVHGSSLWMLCTDVALEFPRPTLPNVVYVGGILTKPAGPLPEDLQRWVNGANEHGFVLVSFGAGVKYLSEDIANKLAGALGRLPQKVIWRFSGTKPKNLGNNTKLIEWLPQNDLLGHSNIKAFLSHGGLNSIFETMYHGVPVVGIPLFGDHYDTMTRVQAKGMGILLEWKTVTEGELYEALVKVINNPSYRQRAQKLSEIHKDQPGHPVNRTVYWIDYILRHNGAHHLRAAVHQISFCQYFLLDIAFVLLLGAALFYFFLSWVTKFIYRKIKSLWSRNKHSTVNGHYHNGILNGKYKRNGHIKHEKKVK

SEQ ID NO: 3 - DNA, 10648 bp, Homo sapiens
  source 1..10648: mol_type = genomic DNA
gtcgagaagcagctacccaagctccaggagcttccggtatgtgttttccctctgttctcgattaccttggcaacggctgaggcgggagaccggtggtctgcaccgtcctggagggagatatgagtggctggactctcagccagccactgggatgtgttcgggctttggaccttgaggccggagagagctcccgagaggaggcggcgccacgttcgttcttctgaggggacggtagatttgggggttttcctctaggattctcgcgccgtttcctctggtaggaacgtcttctgtgttctgattgtttttctaagctgggttcagatgctgtcctttttatgagttttccctacaatcctgcactatcttccttcgctcctcctcgcctccttcccctagcgccccaatctctcttacacctcccggcacatctttcttctcgatctgattacctcctacgtcctctttctcctcgatctggttaccgcctaccattttcacctccgagaggcctcttctgacttccaggctggatcagggccctcgaatttccctgggtcgtagaaaagcgatcattctcttgtcacagactatgcgccttggggccgagaccagaattcacctatttttagcttcagcgtaggggagactagtgcgaagaccactgatttgggagtcaggagccctccagagtcaggttttgcaaattctcagctgtgtgaccctgattctaccttatagagtttgattcctcctctatatggttgttttagagagttcatgagaggaggctctgtgggcggggggggggtgggtctttgtaaagtgtcagtacagaagggagtgactgaatgaatttgagagagatgaatctgttatgctgaaaggtaaatacttaacctgggttctctctggcagcaaggaaatgctgtgtggtttgaaaaacgctttgctatttagattgggatcggcctcttgtatgggaactacctgactttatgtaatatgttgtttggtgtgaaagagaccttggcaatcagccaatccactgccctcattttacagaagaaacaggaccagagagggaaggtgacctgaaagtcacagaataattttttagagctgaacaagaatccaagcctgcaactgcagagacgagagatctttctgctgtctatactcttggaaagcacatcctaaggtactttgattttacagtcatctttccctttttattttatgttttgttttgttttgtttgttattgagacatggtctcactccgtcacttaggctggagtgcagtagtgtgaacatggctaactgaagactttcaacctcctgggctcaagtgatcctcttgcctcagccttccgtgtagctcagaccacaggcacccaccaccatgctcagttaatttttttgatttttttttttttttggtagagatagggtttcacctcattgctcagactggtctcaaattcctgggctcaagtgatcctcccatctcagcctcccaaggtgctggccaagaccagaattacaggcatgagccaccgtgcctgaccttccatctttgcctttttaaatactcacccccatggctccccgagtcacagccctccttatactctattgtaattgctttttctcttgtctgtctctttgctaaaatgtcaccttctaaggggcaaaggcttaacttttgttctgtgttcccaacatccagtatagggttaagcttttagttgaagttagctaatgacaacagcaaatgtctcttaggcacacattatacaccaggcatgatagatacaattctaatgaagtctttgcaatgaccacataaggtagcttccattatccccattttacagatgaggaaacagaggcttaggaaggttaagtacctttctgaagatcacagcgggtaagtagcagagccaggatttgaacacagtctgggtgctgagccctgtcccatagctgtgaccctatgctgactcaaggaagtcagcctgtaccgaaataatggctggcaaaggcctttggggatttgagactcagaaaccaattcatttttttcccccagatctttgcagattatcctgtggaaggaaaatgcctaaagtcaaaagaagccggaaagcacccccagatggctgggagttgattgagccaacactggatgaattagatcaaaagatgagagaaggtgagtaggggagttcctgtctgggtgggctgggtccaagggtcacaggcttagatgcccccaggggacaggcataaatgcaaatataaaaagagagtggtctactaacactgacatgttgtgtttgcttatgaacttggggaaatactgtaagtgcccgaaaataagataacattaatgaaaaggtcctcagaaaaggtgtttttttttgtttttgtttttgccaactcgaatataaaaggttatgaaatatagatcaaatagtctacctatagttatttactattttggttagatatatatttaaaatcatacaaaatatatttacttggaagtgctattccttttcagtatcatcgattagtctttgccgcatctgttttctgtcacttccttgtaaatggcgtgtgatcctgctttgtgaacccgtgtcctatgctgtctttggaaattttatctgaagccacaagcatctgttggccttatatgatcacagtgtggccacttaccaattgacttttttatttttattttttgagttggagtcttgctctgtcttccaggctgcagtgcagtggcgtgatctcggctcactgcaacctctgcctcccgtgttcaagtgattttcctgcctctcagcctctcgagtaatttggattacaggcatgcgccaccatgcccggctaatttttgtatttttagtagagatgggtttctccatgttggccaggctggtctcgaactcctggcctcaagtgatccacccacctcggcctcccaaagtgatgggattacaggtatgagccactacacccagctgaagttactttttaaagtagcttttgaaatgcttgcttgtaactaacctaatcatggttattatgaggtcgtacctccagcagtaattactaaattaaatcaatgttaaattactttgcccctttttaaaaaaactgttcgtaccagataacttctattaaatactcagtacttgttttgcagtttagatttggatgggcctattgcagtaatcacggtcattttgggctgagagatgtcttcccgaaacagctctttatcaaaataaaggaaatgggagcatgctggaatagaagagattttgcaagtccttgaaagtaaattaacttcatcttctaaagggtgacttttgagggaaggaggaaccctactttgtgtttagatattctttacctccagacagaagtattctttgttctgttttctttttgtttttgttttgagacaaggtctcactttgttgcccaggctggagtgcagtggttcaatcacagctcactgaagcctccacctcccaggctcaggtgttcctcccacctcagtctcccaggcagctgggactacaggcatccactgccacgcttggctaagttttcttttcttttttttcttttttttttttttgagacggagtctcgctctgtcacccaggctggagtgcagtggcgcgatctccgctcactgcaagctccgcctcccaggtccacaccattctcctgcctcagcctctggagtagctgggactacaggcgcccgccaccatgcccagctaattttttttttttttttgtatttttagtagagacggggtttcaccatgttagccaggatggtctcgatcgcctgaccttgtgatccacccgcctcaggctcccaaagtgctaggattacaagcatgagccaccgcgcccgaccaacgcttggctaattttttgtagagatgggggtgtgttagtccattttcacgctactgatagacatacctgagactgggcaatttacgaaagaacgagatctaatggacttaccgttccatgtggttggagaggcctcaccatcatggcagaggccaaggaggagcaagtcacgtcttaacatgtgtacctgctgaatctttactacctgcttttctgcttggatcacagcattctgtttgttgagctgaattgtaattcctaggtaatagaatggcttaaaagctggagacagggagggatagtcttcttgaccactcttcgcccttctgttcttccctaaaaactgaggaggtcatagacaaagatgaacttgtgactgctgagagagagagaactgccttgcggcaagtatgagtgccacctgatcctgcgtgtgttgaaggagcagcttctgctgtggctacttccctcagaacctgtagactggtctagtttatttagcttttcctcagccctaaaggactttggctgggagatgaaattagaagtgccttcaagatgattaggatgcccatctgtgggcctagaattatcttgattaattattacgctgtagaaatagatctgaaagcatagggaccaaggttggttttttggcttttttttgtttgttttgttttgtttttttttgagacagggtcatctgtcatccaggctggagtgcagtggcacaatgtcagctaactgcaacctctgcttcccaggttcaagcacttctcgtgcctcagcctcccgagtaactgggattacaggcatgtgccaccatgcccagataatttttgtattttcagtagagacagtgttttgccctgttggccagggtgttctcgaactcctgacctcaagtgatccacccacctcggcctccaaaagtgctgggattacaggcgtgagccactgtgcccagccgggaccaaccttttaacagaagttaccattaaatgtctttaaaaatctatgttttctaattctgtaattaaaaagactttttttcttgtcacatgggtaatgtgccaacgttgtgacaaggtttgagagtggcatgtctcacacatggatgtgaacacccaagcacactcatgaattacaaaaggatccaaaaatagacatttttaatttaaaacaattatgtttaaattacttagcttattttttatttttttatttttttttttgagacggaatctcacactgttgcccacgctggagtgcagtggtgcgatcttggctcactgcaacctgtacctcccgagttcaggcaattctcctgcctcagcctcttgagaagctgggattacaagcgtgcactaccacgcccggctaattttttaatttttagtagtgatggggtttcaccacgttggtcaggctgatctcgatctcctgacctcgtggtccgcccaccttggcctcccaaaatgcccggcggcttattctgtttttaaataacagctttattgagatattaatcatatactgtaaaagtgaacctgttaaattatccaattaaggggtttttagtatattcacaaagttgtacgaccattgccacagttagtttgatgtttcaaggttcatctgtgttgtagaatatatcagtacttacttcattcccttttttttctttttttgagacgggagtcttgctttgttgcctaggctggagtgcagtggtgtgatctcagctcactgcatcctccgcctctgggttcaaacgattctcccacctcagcctcccaagtaggtgggattacaggcatgcgccaccatgccctgctaattcttttgtatttttagtagagatggggtttcaccatgttgaccaagctggtctcagactcctgacctcaagtgacctgcccacctcagcctcccaaagtgctgggattacaggtgtgagccaccgattccggccagccctgtttaacttcttgaggagccacctaactcttctgcagtggctccaccattttacattcccaccaggaacgtaggagagttccaatttctccacatccttcccaacacttgttattgtgccataattttgattatagtcatctgtagggtccagccccacagggtcggtgggtttctccccgtgtgtggagacgagagagcgtagaaataaagacacaagacaaagagataaaagacagctgagcctgggaatcccaccaagacgcggagaccggtagtggccccaaatgccaggctgcactgatatttattggatacaagacaaaggggcaggataagcagtgtgaaccatctccaatgataggtaaggccacatgggtcacgtgtccactggaaagcgggcccttgcctgcctggcaccaaggcagagagagagagacagcttatgccattatttctgcttatcagagacttttagtactttcactaatttgctattgttatctaaaaggcagagccaggtgtacaggatggaacatgaaggcggactaggagcgtgaccaccaaagcacagcatcacagggagatagttaggcctctggataactgcgggcgggcctgactgatgtcaggccctccacaagaggtggaggagtagagtcttctctaaactcccccggggaaagggagattccctttcccggtctgctaagtagcgggtgtttttccttgacactaacgctactgctagaccaaggtccgcttggcaacgggcatcttcccagatgctggcgttaccgctagaccaaggagccctctggtggccctgtccgggcataacagaaggcttgcactcgttttctggtcagttctcactatgtcccctcagctcccatctctgtatagcctggtgtttcctaggttatgattgtcgagtgaggattattataatattggaataaagagtaattgctacaaactaaggattaatgatattcatatataatcatatctaagatctatatctagtataactattcttattttatttattttattatactagaacagctcgtgccctcggtttcttgcctcggcacctgggtggcttgccacccacagccatcctagtgggtataaagtggtatttattcattatcagtagttacttacaaaaagaaaatcctgcgcagaccgaccctattcccccaaacacactctttgtttctccccagctgaaacagaaccgcatgagggaaagaggaaagtggaatctctgtggcccatcttcaggatccaccaccagaaaacccgctacatcttcgacctcttttacaagcggaaagccatcagcagaggtaattagtcagtctctcttggactttgaagctcgcgtcacttttggagttactgaactaaccacaatccttattctcgcaacctgtgcaagtcatggtttttcttaccacgaaaattagggggagccaacgttggctgagttttgtgtgtgtgtttgttttttgtttgtttgttttgagatggagtctcactctgtcacccaggctggagtgcagtggcgcaatcttggctcactgcaagctccacttcctgggttcaagcgattctcctgtctcagctcccaagtagctgggattacaggcacctgccaccacacctggccaatttttgtatttttagtaaagatggggtttcaccatattggtcaggctgatcttgaactcctgacctcaggtgattcacccgactcggtctcccaaagtgctggaattataggcgtggtccaccgctcttggctttttttttttttttttttttgaaacagggtcttgctctgttccacaggctggagtgcagtggtgcaatgatggctcactgcagcctcaaccttctgggctcaagggatcctctcacctcaacctcctgagtagctgtgactacaggtgtgcaccaccacacccagctaatttttaaattttttgtggagatgggcccttggcccaggctggtttcttaactcaaatgatcctctggcgttggcttccaaaagtgctgggattacaggtgtgaggcaccttgcctggcctaagtactttttttttttgttcctcctccaaggactgtcccgttgcaatactgaatgcctttttttttttgagatggagtttcgctgtcacccaggctggagtccagtggcacgacctcaggtcactacaacctccgcctcctgggttcaagtgattctcctgcctcagcctcctaagtagctgggattacagctgctaccacgcccgagtaatttttgtatttttagtagagacggggttttaccatgttggccgggctggtcctgaactcctgacctcaggtgatccgcctgcctcggcctcccaaagtgctgggattacaggtgtgagccactgcacccggcctgaatgctttttttgatcaagggtggggaaggtttttagaccatggcctgatgctctttccccatctttttgacagaactctatgaatattgtattaaagaaggctatgcagacaaaaacctgattgcaaaatggaaaaagcaaggatatgagaacttgtgctgcctgcggtgcattcagacacgggacaccaacttcgggacgaactgcatctgccgcgtgcccaaaagcaagctggaagtggtaatgtctgacactcaagcttggtgttgttttcagctcaaaattctgccttagtcgactgcaagggatcttatgttatttggttgggctggaatgtcgttttgtccctggatgtcctgctggctctccctcgtgggagtgggtccctgtattcaggaatccatgtgaggcagcgtgtggctgtgtgtttgttaggtctggggtcaatctcaactccacttttgggcaaattactgaacccctttcctcacttaggaaatggtggtggggagccctaatcccaaggtggtggcagggtgacatcagggaaggacaaccagtgagttcctgtccctttcagtcctcacagtgatactttaacattaccatcactatctttcccgcccccccaagacggagtcttgctttgtcgcccaggctggagtgcagtgatgccatcttggctcactgcaacctccacctcccgggttcaagcggttctcctgcctcatcctcctgagtagctgggactacaggcatgcaccaccacgcctggctaattttgtatttttagtagagacggggtttctcaatgttgctcaggctggtctcgaactcccgacctcaggtgatccacccgcctcagcctcccaaagtgccgggattacaggcatgagctactgcgcccagcccactgtgtttcttctttcagaactttctgttccaagtaccactcctaggccaggcgcctcaggagtggtgctgagggacaggagctgagctccatccggttccaagcccctctgaaaggcagctgtggcccgaggcagagtcacagcagtggccgctcagtgcagcccctcagcacagttgttggccccaccgcccatctgccagcctggccttcttttccccagctccacacaggggcctcttcacatgagtcccctttatgctgcagtgagactgacaatggagagctgtggctggatgctgaggacttgggtactgagcagtgggggcgagcaagggccgcctccccgacggaagactggggtgttggttttctgatggaggcagggacaggtggcagagtggcagaagcccccttcctctgagtgcccagattccacaaggagtccaggtcaggggctggtgggctggggtgctgcttcagccctgtggccaaaacagcccgctgtagacttacctgggtttcaccagaggatcctgtttacttaaactatggtcttgttcttccaaaaaaagaacttgaaaaagtaaaataaacacaagccactgttctagggctttctggctggccaagtgttgggccgcaccaggcctgggggacaagacccttctttctggggggctctgggccagaagggtgtgactcaagtgcatagtctcctgccctcttcccccaccagagtgtaccagcccagaggcccccctgaagtccccaaacagtagcagagccacgtctgctcatcgcagggtctgtcatgctcacttagcagaataacgagactcattcacaccgatttctttttcttgattggcaaacgtgtgttggatttgcagaacatattataaatagacatacagatgtaacctcggtgtcaacagcagctggttctaccttcatgagggagccaaattttccctgtccagagctgtcaaggaagggtttctgaggtgtgtccctatatggcatggtggcaggtccttcgtgggagggttgccacatatgtgagtgtgcaggggcgagcgtggcgcagtggcatcgtctcactgtcctcctccgttgcagggccgcatcatcgagtgcacacactgtggctgtcgtggctgctctggctgaggctggcgcgctccaccctggactctggacttcgcaggttcctgcctgtcacgccacccccttcctgggagcagcgagcagtgccccaggcccgagttggagcacggtctctatggggaaggcttcgctgtctatcagctgtgatttgtaaaaataaaatctttaaatctctcga

SEQ ID NO: 4 - protein, 144 aa, synthetic construct
MPKVKRSRKAPPDGWELIEPTLDELDQKMREAETEPHEGKRKVESLWPIFRIHHQKTRYIFDLFYKRKAISRELYEYCIKEGYADKNLIAKWKKQGYENLCCLRCIQTRDTNFGTNCICRVPKSKLEVGRIIECTHCGCRGCSG